European Patent Application EP 4 772 635 A1, published July 8, 2026. Title: RNAI AGENT TARGETING APP AND PHARMACEUTICAL USE THEREOF. Applicant: TUOJIE BIOTECH (SHANGHAI) CO., LTD. Application WO. The sequence listing filed with the application follows.

SEQUENCE LISTING (250 sequences)

SEQ ID NO: 1 - RNA, 19 nt, Synthetic Construct
  source 1..19: mol_type = other RNA; note = unmodified sense strand
agtctaccctgaactgcag

SEQ ID NO: 2 - RNA, 19 nt, Synthetic Construct
  source 1..19: mol_type = other RNA; note = unmodified sense strand
agtctaccctgaactgcaa

SEQ ID NO: 3 - RNA, 19 nt, Synthetic Construct
  source 1..19: mol_type = other RNA; note = unmodified sense strand
tgacgaggacgatgaggat

SEQ ID NO: 4 - RNA, 19 nt, Synthetic Construct
  source 1..19: mol_type = other RNA; note = unmodified sense strand
tgacgaggacgatgaggaa

SEQ ID NO: 5 - RNA, 19 nt, Synthetic Construct
  source 1..19: mol_type = other RNA; note = unmodified sense strand
gaacgtgggagttcagcta

SEQ ID NO: 6 - RNA, 19 nt, Synthetic Construct
  source 1..19: mol_type = other RNA; note = unmodified sense strand
ttaagtatttcagatgctt

SEQ ID NO: 7 - RNA, 19 nt, Synthetic Construct
  source 1..19: mol_type = other RNA; note = unmodified sense strand
ttaagtatttcagatgcta

SEQ ID NO: 8 - RNA, 19 nt, Synthetic Construct
  source 1..19: mol_type = other RNA; note = unmodified sense strand
ggggtgctctgctggtctt

SEQ ID NO: 9 - RNA, 19 nt, Synthetic Construct
  source 1..19: mol_type = other RNA; note = unmodified sense strand
ggggtgctctgctggtcta

SEQ ID NO: 10 - RNA, 19 nt, Synthetic Construct
  source 1..19: mol_type = other RNA; note = unmodified sense strand
ggtgctctgctggtcttca

SEQ ID NO: 11 - RNA, 19 nt, Synthetic Construct
  source 1..19: mol_type = other RNA; note = unmodified sense strand
gtgctctgctggtcttcaa

SEQ ID NO: 12 - RNA, 21 nt, Synthetic Construct
  source 1..21: mol_type = other RNA; note = unmodified anti-sense strand
ctgcagttcagggtagacttc

SEQ ID NO: 13 - RNA, 21 nt, Synthetic Construct
  source 1..21: mol_type = other RNA; note = unmodified anti-sense strand
ttgcagttcagggtagacttc

SEQ ID NO: 14 - RNA, 21 nt, Synthetic Construct
  source 1..21: mol_type = other RNA; note = unmodified anti-sense strand
atcctcatcgtcctcgtcatc

SEQ ID NO: 15 - RNA, 21 nt, Synthetic Construct
  source 1..21: mol_type = other RNA; note = unmodified anti-sense strand
ttcctcatcgtcctcgtcatc

SEQ ID NO: 16 - RNA, 21 nt, Synthetic Construct
  source 1..21: mol_type = other RNA; note = unmodified anti-sense strand
tagctgaactcccacgttcac

SEQ ID NO: 17 - RNA, 21 nt, Synthetic Construct
  source 1..21: mol_type = other RNA; note = unmodified anti-sense strand
aagcatctgaaatacttaaaa

SEQ ID NO: 18 - RNA, 21 nt, Synthetic Construct
  source 1..21: mol_type = other RNA; note = unmodified anti-sense strand
tagcatctgaaatacttaaaa

SEQ ID NO: 19 - RNA, 21 nt, Synthetic Construct
  source 1..21: mol_type = other RNA; note = unmodified anti-sense strand
aagaccagcagagcacccctc

SEQ ID NO: 20 - RNA, 21 nt, Synthetic Construct
  source 1..21: mol_type = other RNA; note = unmodified anti-sense strand
tagaccagcagagcacccctc

SEQ ID NO: 21 - RNA, 21 nt, Synthetic Construct
  source 1..21: mol_type = other RNA; note = unmodified anti-sense strand
tgaagaccagcagagcacccc

SEQ ID NO: 22 - RNA, 21 nt, Synthetic Construct
  source 1..21: mol_type = other RNA; note = unmodified anti-sense strand
ttgaagaccagcagagcaccc

SEQ ID NO: 23 - RNA, 19 nt, Synthetic Construct
  source 1..19: mol_type = other RNA; note = unmodified sense strand
cgaggacgatgaggatggt

SEQ ID NO: 24 - RNA, 19 nt, Synthetic Construct
  source 1..19: mol_type = other RNA; note = unmodified sense strand
ggacgatgaggatggtgat

SEQ ID NO: 25 - RNA, 19 nt, Synthetic Construct
  source 1..19: mol_type = other RNA; note = unmodified sense strand
cgatgaggatggtgatgaa

SEQ ID NO: 26 - RNA, 19 nt, Synthetic Construct
  source 1..19: mol_type = other RNA; note = unmodified sense strand
ggctgaggaaccctacgaa

SEQ ID NO: 27 - RNA, 19 nt, Synthetic Construct
  source 1..19: mol_type = other RNA; note = unmodified sense strand
gctgaggaaccctacgaaa

SEQ ID NO: 28 - RNA, 19 nt, Synthetic Construct
  source 1..19: mol_type = other RNA; note = unmodified sense strand
ctgaggaaccctacgaaga

SEQ ID NO: 29 - RNA, 19 nt, Synthetic Construct
  source 1..19: mol_type = other RNA; note = unmodified sense strand
tgaggaaccctacgaagaa

SEQ ID NO: 30 - RNA, 19 nt, Synthetic Construct
  source 1..19: mol_type = other RNA; note = unmodified sense strand
gaggaaccctacgaagaaa

SEQ ID NO: 31 - RNA, 19 nt, Synthetic Construct
  source 1..19: mol_type = other RNA; note = unmodified sense strand
gaaccctacgaagaagcca

SEQ ID NO: 32 - RNA, 19 nt, Synthetic Construct
  source 1..19: mol_type = other RNA; note = unmodified sense strand
accctacgaagaagccaca

SEQ ID NO: 33 - RNA, 19 nt, Synthetic Construct
  source 1..19: mol_type = other RNA; note = unmodified sense strand
cctacgaagaagccacaga

SEQ ID NO: 34 - RNA, 19 nt, Synthetic Construct
  source 1..19: mol_type = other RNA; note = unmodified sense strand
tacgaagaagccacagaga

SEQ ID NO: 35 - RNA, 19 nt, Synthetic Construct
  source 1..19: mol_type = other RNA; note = unmodified sense strand
cgaagaagccacagagaga

SEQ ID NO: 36 - RNA, 19 nt, Synthetic Construct
  source 1..19: mol_type = other RNA; note = unmodified sense strand
gaagaagccacagagagaa

SEQ ID NO: 37 - RNA, 19 nt, Synthetic Construct
  source 1..19: mol_type = other RNA; note = unmodified sense strand
gaagccacagagagaacca

SEQ ID NO: 38 - RNA, 19 nt, Synthetic Construct
  source 1..19: mol_type = other RNA; note = unmodified sense strand
gccacagagagaaccacca

SEQ ID NO: 39 - RNA, 19 nt, Synthetic Construct
  source 1..19: mol_type = other RNA; note = unmodified sense strand
ccacagagagaaccaccaa

SEQ ID NO: 40 - RNA, 19 nt, Synthetic Construct
  source 1..19: mol_type = other RNA; note = unmodified sense strand
gccaccaccaccaccacca

SEQ ID NO: 41 - RNA, 19 nt, Synthetic Construct
  source 1..19: mol_type = other RNA; note = unmodified sense strand
gagaggtgtgctctgaaca

SEQ ID NO: 42 - RNA, 19 nt, Synthetic Construct
  source 1..19: mol_type = other RNA; note = unmodified sense strand
agaggtgtgctctgaacaa

SEQ ID NO: 43 - RNA, 19 nt, Synthetic Construct
  source 1..19: mol_type = other RNA; note = unmodified sense strand
ggccgtgccgagcaatgat

SEQ ID NO: 44 - RNA, 19 nt, Synthetic Construct
  source 1..19: mol_type = other RNA; note = unmodified sense strand
ccgtgccgagcaatgatct

SEQ ID NO: 45 - RNA, 19 nt, Synthetic Construct
  source 1..19: mol_type = other RNA; note = unmodified sense strand
cgtgccgagcaatgatcta

SEQ ID NO: 46 - RNA, 19 nt, Synthetic Construct
  source 1..19: mol_type = other RNA; note = unmodified sense strand
ggatgtggcggcaaccgga

SEQ ID NO: 47 - RNA, 19 nt, Synthetic Construct
  source 1..19: mol_type = other RNA; note = unmodified sense strand
gatgtggcggcaaccggaa

SEQ ID NO: 48 - RNA, 19 nt, Synthetic Construct
  source 1..19: mol_type = other RNA; note = unmodified sense strand
ggcggcaaccggaacaact

SEQ ID NO: 49 - RNA, 19 nt, Synthetic Construct
  source 1..19: mol_type = other RNA; note = unmodified sense strand
gcggcaaccggaacaactt

SEQ ID NO: 50 - RNA, 19 nt, Synthetic Construct
  source 1..19: mol_type = other RNA; note = unmodified sense strand
cggcaaccggaacaacttt

SEQ ID NO: 51 - RNA, 19 nt, Synthetic Construct
  source 1..19: mol_type = other RNA; note = unmodified sense strand
ggcaaccggaacaacttta

SEQ ID NO: 52 - RNA, 19 nt, Synthetic Construct
  source 1..19: mol_type = other RNA; note = unmodified sense strand
gcaaccggaacaactttga

SEQ ID NO: 53 - RNA, 19 nt, Synthetic Construct
  source 1..19: mol_type = other RNA; note = unmodified sense strand
agaacgtcaagcaaagaaa

SEQ ID NO: 54 - RNA, 19 nt, Synthetic Construct
  source 1..19: mol_type = other RNA; note = unmodified sense strand
ggccagagtggaagccata

SEQ ID NO: 55 - RNA, 19 nt, Synthetic Construct
  source 1..19: mol_type = other RNA; note = unmodified sense strand
agaacagaaggacagacaa

SEQ ID NO: 56 - RNA, 19 nt, Synthetic Construct
  source 1..19: mol_type = other RNA; note = unmodified sense strand
tcacatagccccttagcca

SEQ ID NO: 57 - RNA, 19 nt, Synthetic Construct
  source 1..19: mol_type = other RNA; note = unmodified sense strand
gccccttagccagttgtat

SEQ ID NO: 58 - RNA, 19 nt, Synthetic Construct
  source 1..19: mol_type = other RNA; note = unmodified sense strand
ccccttagccagttgtata

SEQ ID NO: 59 - RNA, 19 nt, Synthetic Construct
  source 1..19: mol_type = other RNA; note = unmodified sense strand
atgtgaacgtgggagttca

SEQ ID NO: 60 - RNA, 19 nt, Synthetic Construct
  source 1..19: mol_type = other RNA; note = unmodified sense strand
taagtatttcagatgcttt

SEQ ID NO: 61 - RNA, 19 nt, Synthetic Construct
  source 1..19: mol_type = other RNA; note = unmodified sense strand
ggaattaagaggatacaca

SEQ ID NO: 62 - RNA, 19 nt, Synthetic Construct
  source 1..19: mol_type = other RNA; note = unmodified sense strand
gaattaagaggatacacaa

SEQ ID NO: 63 - RNA, 19 nt, Synthetic Construct
  source 1..19: mol_type = other RNA; note = unmodified sense strand
gcattgagacttcaagctt

SEQ ID NO: 64 - RNA, 19 nt, Synthetic Construct
  source 1..19: mol_type = other RNA; note = unmodified sense strand
cattgagacttcaagcttt

SEQ ID NO: 65 - RNA, 19 nt, Synthetic Construct
  source 1..19: mol_type = other RNA; note = unmodified sense strand
ggaggggtgctctgctggt

SEQ ID NO: 66 - RNA, 21 nt, Synthetic Construct
  source 1..21: mol_type = other RNA; note = unmodified anti-sense strand
accatcctcatcgtcctcgtc

SEQ ID NO: 67 - RNA, 21 nt, Synthetic Construct
  source 1..21: mol_type = other RNA; note = unmodified anti-sense strand
atcaccatcctcatcgtcctc

SEQ ID NO: 68 - RNA, 21 nt, Synthetic Construct
  source 1..21: mol_type = other RNA; note = unmodified anti-sense strand
ttcatcaccatcctcatcgtc

SEQ ID NO: 69 - RNA, 21 nt, Synthetic Construct
  source 1..21: mol_type = other RNA; note = unmodified anti-sense strand
ttcgtagggttcctcagcctc

SEQ ID NO: 70 - RNA, 21 nt, Synthetic Construct
  source 1..21: mol_type = other RNA; note = unmodified anti-sense strand
tttcgtagggttcctcagcct

SEQ ID NO: 71 - RNA, 21 nt, Synthetic Construct
  source 1..21: mol_type = other RNA; note = unmodified anti-sense strand
tcttcgtagggttcctcagcc

SEQ ID NO: 72 - RNA, 21 nt, Synthetic Construct
  source 1..21: mol_type = other RNA; note = unmodified anti-sense strand
ttcttcgtagggttcctcagc

SEQ ID NO: 73 - RNA, 21 nt, Synthetic Construct
  source 1..21: mol_type = other RNA; note = unmodified anti-sense strand
tttcttcgtagggttcctcag

SEQ ID NO: 74 - RNA, 21 nt, Synthetic Construct
  source 1..21: mol_type = other RNA; note = unmodified anti-sense strand
tggcttcttcgtagggttcct

SEQ ID NO: 75 - RNA, 21 nt, Synthetic Construct
  source 1..21: mol_type = other RNA; note = unmodified anti-sense strand
tgtggcttcttcgtagggttc

SEQ ID NO: 76 - RNA, 21 nt, Synthetic Construct
  source 1..21: mol_type = other RNA; note = unmodified anti-sense strand
tctgtggcttcttcgtagggt

SEQ ID NO: 77 - RNA, 21 nt, Synthetic Construct
  source 1..21: mol_type = other RNA; note = unmodified anti-sense strand
tctctgtggcttcttcgtagg

SEQ ID NO: 78 - RNA, 21 nt, Synthetic Construct
  source 1..21: mol_type = other RNA; note = unmodified anti-sense strand
tctctctgtggcttcttcgta

SEQ ID NO: 79 - RNA, 21 nt, Synthetic Construct
  source 1..21: mol_type = other RNA; note = unmodified anti-sense strand
ttctctctgtggcttcttcgt

SEQ ID NO: 80 - RNA, 21 nt, Synthetic Construct
  source 1..21: mol_type = other RNA; note = unmodified anti-sense strand
tggttctctctgtggcttctt

SEQ ID NO: 81 - RNA, 21 nt, Synthetic Construct
  source 1..21: mol_type = other RNA; note = unmodified anti-sense strand
tggtggttctctctgtggctt

SEQ ID NO: 82 - RNA, 21 nt, Synthetic Construct
  source 1..21: mol_type = other RNA; note = unmodified anti-sense strand
ttggtggttctctctgtggct

SEQ ID NO: 83 - RNA, 21 nt, Synthetic Construct
  source 1..21: mol_type = other RNA; note = unmodified anti-sense strand
tggtggtggtggtggtggcaa

SEQ ID NO: 84 - RNA, 21 nt, Synthetic Construct
  source 1..21: mol_type = other RNA; note = unmodified anti-sense strand
tgttcagagcacacctctcga

SEQ ID NO: 85 - RNA, 21 nt, Synthetic Construct
  source 1..21: mol_type = other RNA; note = unmodified anti-sense strand
ttgttcagagcacacctctcg

SEQ ID NO: 86 - RNA, 21 nt, Synthetic Construct
  source 1..21: mol_type = other RNA; note = unmodified anti-sense strand
atcattgctcggcacggcccc

SEQ ID NO: 87 - RNA, 21 nt, Synthetic Construct
  source 1..21: mol_type = other RNA; note = unmodified anti-sense strand
agatcattgctcggcacggcc

SEQ ID NO: 88 - RNA, 21 nt, Synthetic Construct
  source 1..21: mol_type = other RNA; note = unmodified anti-sense strand
tagatcattgctcggcacggc

SEQ ID NO: 89 - RNA, 21 nt, Synthetic Construct
  source 1..21: mol_type = other RNA; note = unmodified anti-sense strand
tccggttgccgccacatccgc

SEQ ID NO: 90 - RNA, 21 nt, Synthetic Construct
  source 1..21: mol_type = other RNA; note = unmodified anti-sense strand
ttccggttgccgccacatccg

SEQ ID NO: 91 - RNA, 21 nt, Synthetic Construct
  source 1..21: mol_type = other RNA; note = unmodified anti-sense strand
agttgttccggttgccgccac

SEQ ID NO: 92 - RNA, 21 nt, Synthetic Construct
  source 1..21: mol_type = other RNA; note = unmodified anti-sense strand
aagttgttccggttgccgcca

SEQ ID NO: 93 - RNA, 21 nt, Synthetic Construct
  source 1..21: mol_type = other RNA; note = unmodified anti-sense strand
aaagttgttccggttgccgcc

SEQ ID NO: 94 - RNA, 21 nt, Synthetic Construct
  source 1..21: mol_type = other RNA; note = unmodified anti-sense strand
taaagttgttccggttgccgc

SEQ ID NO: 95 - RNA, 21 nt, Synthetic Construct
  source 1..21: mol_type = other RNA; note = unmodified anti-sense strand
tcaaagttgttccggttgccg

SEQ ID NO: 96 - RNA, 21 nt, Synthetic Construct
  source 1..21: mol_type = other RNA; note = unmodified anti-sense strand
tttctttgcttgacgttctgc

SEQ ID NO: 97 - RNA, 21 nt, Synthetic Construct
  source 1..21: mol_type = other RNA; note = unmodified anti-sense strand
tatggcttccactctggccat

SEQ ID NO: 98 - RNA, 21 nt, Synthetic Construct
  source 1..21: mol_type = other RNA; note = unmodified anti-sense strand
ttgtctgtccttctgttctgc

SEQ ID NO: 99 - RNA, 21 nt, Synthetic Construct
  source 1..21: mol_type = other RNA; note = unmodified anti-sense strand
tggctaaggggctatgtgata

SEQ ID NO: 100 - RNA, 21 nt, Synthetic Construct
  source 1..21: mol_type = other RNA; note = unmodified anti-sense strand
atacaactggctaaggggcta

SEQ ID NO: 101 - RNA, 21 nt, Synthetic Construct
  source 1..21: mol_type = other RNA; note = unmodified anti-sense strand
tatacaactggctaaggggct

SEQ ID NO: 102 - RNA, 21 nt, Synthetic Construct
  source 1..21: mol_type = other RNA; note = unmodified anti-sense strand
tgaactcccacgttcacatga

SEQ ID NO: 103 - RNA, 21 nt, Synthetic Construct
  source 1..21: mol_type = other RNA; note = unmodified anti-sense strand
aaagcatctgaaatacttaaa

SEQ ID NO: 104 - RNA, 21 nt, Synthetic Construct
  source 1..21: mol_type = other RNA; note = unmodified anti-sense strand
tgtgtatcctcttaattccta

SEQ ID NO: 105 - RNA, 21 nt, Synthetic Construct
  source 1..21: mol_type = other RNA; note = unmodified anti-sense strand
ttgtgtatcctcttaattcct

SEQ ID NO: 106 - RNA, 21 nt, Synthetic Construct
  source 1..21: mol_type = other RNA; note = unmodified anti-sense strand
aagcttgaagtctcaatgcct

SEQ ID NO: 107 - RNA, 21 nt, Synthetic Construct
  source 1..21: mol_type = other RNA; note = unmodified anti-sense strand
aaagcttgaagtctcaatgcc

SEQ ID NO: 108 - RNA, 21 nt, Synthetic Construct
  source 1..21: mol_type = other RNA; note = unmodified anti-sense strand
accagcagagcacccctcccc

SEQ ID NO: 109 - RNA, 19 nt, Synthetic Construct
  source 1..19: mol_type = other RNA; note = modified sense strand
  modified_base 1..6: mod_base = OTHER; note = modified with 2'-methoxy
  modified_base 7..9: mod_base = OTHER; note = modified with 2'-Fluoro
  modified_base 10..19: mod_base = OTHER; note = modified with 2'-methoxy
  modified_base 1..3: mod_base = OTHER; note = two adjacent nucleosides are linked by phosphorothioate diester groups
agtctaccctgaactgcaa

SEQ ID NO: 110 - RNA, 19 nt, Synthetic Construct
  source 1..19: mol_type = other RNA; note = modified sense strand
  modified_base 1..6: mod_base = OTHER; note = modified with 2'-methoxy
  modified_base 7..9: mod_base = OTHER; note = modified with 2'-Fluoro
  modified_base 10..19: mod_base = OTHER; note = modified with 2'-methoxy
  modified_base 1..3: mod_base = OTHER; note = two adjacent nucleosides are linked by phosphorothioate diester groups
tgacgaggacgatgaggaa

SEQ ID NO: 111 - RNA, 19 nt, Synthetic Construct
  source 1..19: mol_type = other RNA; note = modified sense strand
  modified_base 1..6: mod_base = OTHER; note = modified with 2'-methoxy
  modified_base 7..9: mod_base = OTHER; note = modified with 2'-Fluoro
  modified_base 10..19: mod_base = OTHER; note = modified with 2'-methoxy
  modified_base 1..3: mod_base = OTHER; note = two adjacent nucleosides are linked by phosphorothioate diester groups
gaacgtgggagttcagcta

SEQ ID NO: 112 - RNA, 19 nt, Synthetic Construct
  source 1..19: mol_type = other RNA; note = modified sense strand
  modified_base 1..6: mod_base = OTHER; note = modified with 2'-methoxy
  modified_base 7..9: mod_base = OTHER; note = modified with 2'-Fluoro
  modified_base 10..19: mod_base = OTHER; note = modified with 2'-methoxy
  modified_base 1..3: mod_base = OTHER; note = two adjacent nucleosides are linked by phosphorothioate diester groups
ttaagtatttcagatgcta

SEQ ID NO: 113 - RNA, 19 nt, Synthetic Construct
  source 1..19: mol_type = other RNA; note = modified sense strand
  modified_base 1..6: mod_base = OTHER; note = modified with 2'-methoxy
  modified_base 7..9: mod_base = OTHER; note = modified with 2'-Fluoro
  modified_base 10..19: mod_base = OTHER; note = modified with 2'-methoxy
  modified_base 1..3: mod_base = OTHER; note = two adjacent nucleosides are linked by phosphorothioate diester groups
ggggtgctctgctggtcta

SEQ ID NO: 114 - RNA, 19 nt, Synthetic Construct
  source 1..19: mol_type = other RNA; note = modified sense strand
  modified_base 1..6: mod_base = OTHER; note = modified with 2'-methoxy
  modified_base 7..9: mod_base = OTHER; note = modified with 2'-Fluoro
  modified_base 10..19: mod_base = OTHER; note = modified with 2'-methoxy
  modified_base 1..3: mod_base = OTHER; note = two adjacent nucleosides are linked by phosphorothioate diester groups
ggtgctctgctggtcttca

SEQ ID NO: 115 - RNA, 19 nt, Synthetic Construct
  source 1..19: mol_type = other RNA; note = modified sense strand
  modified_base 1..6: mod_base = OTHER; note = modified with 2'-methoxy
  modified_base 7..9: mod_base = OTHER; note = modified with 2'-Fluoro
  modified_base 10..19: mod_base = OTHER; note = modified with 2'-methoxy
  modified_base 1..3: mod_base = OTHER; note = two adjacent nucleosides are linked by phosphorothioate diester groups
gtgctctgctggtcttcaa

SEQ ID NO: 116 - RNA, 19 nt, Synthetic Construct
  source 1..19: mol_type = other RNA; note = modified sense strand
  modified_base 1..6: mod_base = OTHER; note = modified with 2'-methoxy
  modified_base 7..9: mod_base = OTHER; note = modified with 2'-Fluoro
  modified_base 10..19: mod_base = OTHER; note = modified with 2'-methoxy
  modified_base 1..3: mod_base = OTHER; note = two adjacent nucleosides are linked by phosphorothioate diester groups
  modified_base 17..19: mod_base = OTHER; note = two adjacent nucleosides are linked by phosphorothioate diester groups
  modified_base 1: mod_base = OTHER; note = -O-n-hexadecyl is connected at 2' position of the sugar ring
agtctaccctgaactgcaa

SEQ ID NO: 117 - RNA, 19 nt, Synthetic Construct
  source 1..19: mol_type = other RNA; note = modified sense strand
  modified_base 1..6: mod_base = OTHER; note = modified with 2'-methoxy
  modified_base 7..9: mod_base = OTHER; note = modified with 2'-Fluoro
  modified_base 10..19: mod_base = OTHER; note = modified with 2'-methoxy
  modified_base 1..3: mod_base = OTHER; note = two adjacent nucleosides are linked by phosphorothioate diester groups
  modified_base 17..19: mod_base = OTHER; note = two adjacent nucleosides are linked by phosphorothioate diester groups
  modified_base 1: mod_base = OTHER; note = -O-n-hexadecyl is connected at 2' position of the sugar ring
tgacgaggacgatgaggaa

SEQ ID NO: 118 - RNA, 19 nt, Synthetic Construct
  source 1..19: mol_type = other RNA; note = modified sense strand
  modified_base 1..6: mod_base = OTHER; note = modified with 2'-methoxy
  modified_base 7..9: mod_base = OTHER; note = modified with 2'-Fluoro
  modified_base 10..19: mod_base = OTHER; note = modified with 2'-methoxy
  modified_base 1..3: mod_base = OTHER; note = two adjacent nucleosides are linked by phosphorothioate diester groups
  modified_base 17..19: mod_base = OTHER; note = two adjacent nucleosides are linked by phosphorothioate diester groups
  modified_base 1: mod_base = OTHER; note = -O-n-hexadecyl is connected at 2' position of the sugar ring
gaacgtgggagttcagcta

SEQ ID NO: 119 - RNA, 19 nt, Synthetic Construct
  source 1..19: mol_type = other RNA; note = modified sense strand
  modified_base 1..6: mod_base = OTHER; note = modified with 2'-methoxy
  modified_base 7..9: mod_base = OTHER; note = modified with 2'-Fluoro
  modified_base 10..19: mod_base = OTHER; note = modified with 2'-methoxy
  modified_base 1..3: mod_base = OTHER; note = two adjacent nucleosides are linked by phosphorothioate diester groups
  modified_base 17..19: mod_base = OTHER; note = two adjacent nucleosides are linked by phosphorothioate diester groups
  modified_base 1: mod_base = OTHER; note = -O-n-hexadecyl is connected at 2' position of the sugar ring
ttaagtatttcagatgcta

SEQ ID NO: 120 - RNA, 19 nt, Synthetic Construct
  source 1..19: mol_type = other RNA; note = modified sense strand
  modified_base 1..6: mod_base = OTHER; note = modified with 2'-methoxy
  modified_base 7..9: mod_base = OTHER; note = modified with 2'-Fluoro
  modified_base 10..19: mod_base = OTHER; note = modified with 2'-methoxy
  modified_base 1..3: mod_base = OTHER; note = two adjacent nucleosides are linked by phosphorothioate diester groups
  modified_base 17..19: mod_base = OTHER; note = two adjacent nucleosides are linked by phosphorothioate diester groups
  modified_base 1: mod_base = OTHER; note = -O-n-hexadecyl is connected at 2' position of the sugar ring
ggggtgctctgctggtcta

SEQ ID NO: 121 - RNA, 19 nt, Synthetic Construct
  source 1..19: mol_type = other RNA; note = modified sense strand
  modified_base 1..6: mod_base = OTHER; note = modified with 2'-methoxy
  modified_base 7..9: mod_base = OTHER; note = modified with 2'-Fluoro
  modified_base 10..19: mod_base = OTHER; note = modified with 2'-methoxy
  modified_base 1..3: mod_base = OTHER; note = two adjacent nucleosides are linked by phosphorothioate diester groups
  modified_base 17..19: mod_base = OTHER; note = two adjacent nucleosides are linked by phosphorothioate diester groups
  modified_base 1: mod_base = OTHER; note = -O-n-hexadecyl is connected at 2' position of the sugar ring
ggtgctctgctggtcttca

SEQ ID NO: 122 - RNA, 19 nt, Synthetic Construct
  source 1..19: mol_type = other RNA; note = modified sense strand
  modified_base 1..6: mod_base = OTHER; note = modified with 2'-methoxy
  modified_base 7..9: mod_base = OTHER; note = modified with 2'-Fluoro
  modified_base 10..19: mod_base = OTHER; note = modified with 2'-methoxy
  modified_base 1..3: mod_base = OTHER; note = two adjacent nucleosides are linked by phosphorothioate diester groups
  modified_base 17..19: mod_base = OTHER; note = two adjacent nucleosides are linked by phosphorothioate diester groups
  modified_base 1: mod_base = OTHER; note = -O-n-hexadecyl is connected at 2' position of the sugar ring
gtgctctgctggtcttcaa

SEQ ID NO: 123 - RNA, 19 nt, Synthetic Construct
  source 1..19: mol_type = other RNA; note = modified sense strand
  modified_base 1..6: mod_base = OTHER; note = modified with 2'-methoxy
  modified_base 7..9: mod_base = OTHER; note = modified with 2'-Fluoro
  modified_base 10..19: mod_base = OTHER; note = modified with 2'-methoxy
  modified_base 1..3: mod_base = OTHER; note = two adjacent nucleosides are linked by phosphorothioate diester groups
  modified_base 17..19: mod_base = OTHER; note = two adjacent nucleosides are linked by phosphorothioate diester groups
  modified_base 6: mod_base = OTHER; note = -CH2O-n-hexadecyl is connected at 2' position of the sugar ring
ttaagtatttcagatgcta

SEQ ID NO: 124 - RNA, 19 nt, Synthetic Construct
  source 1..19: mol_type = other RNA; note = modified sense strand
  modified_base 1..6: mod_base = OTHER; note = modified with 2'-methoxy
  modified_base 7..9: mod_base = OTHER; note = modified with 2'-Fluoro
  modified_base 10..19: mod_base = OTHER; note = modified with 2'-methoxy
  modified_base 1..3: mod_base = OTHER; note = two adjacent nucleosides are linked by phosphorothioate diester groups
  modified_base 17..19: mod_base = OTHER; note = two adjacent nucleosides are linked by phosphorothioate diester groups
  modified_base 1: mod_base = OTHER; note = -CH2O-n-hexadecyl is connected at 2' position of the sugar ring
ttaagtatttcagatgcta

SEQ ID NO: 125 - RNA, 19 nt, Synthetic Construct
  source 1..19: mol_type = other RNA; note = modified sense strand
  modified_base 1..6: mod_base = OTHER; note = modified with 2'-methoxy
  modified_base 7..9: mod_base = OTHER; note = modified with 2'-Fluoro
  modified_base 10..19: mod_base = OTHER; note = modified with 2'-methoxy
  modified_base 1..3: mod_base = OTHER; note = two adjacent nucleosides are linked by phosphorothioate diester groups
  modified_base 17..19: mod_base = OTHER; note = two adjacent nucleosides are linked by phosphorothioate diester groups
  modified_base 1: mod_base = OTHER; note = -O-n-hexadecyl is connected at 2' position of the sugar ring
ttaagtatttcagatgcta

SEQ ID NO: 126 - RNA, 21 nt, Synthetic Construct
  source 1..21: mol_type = other RNA; note = modified anti-sense strand
  modified_base 1: mod_base = OTHER; note = modified with 2'-methoxy
  modified_base 2: mod_base = OTHER; note = modified with 2'-Fluoro
  modified_base 3..5: mod_base = OTHER; note = modified with 2'-methoxy
  modified_base 6: mod_base = OTHER; note = modified with 2'-Fluoro
  modified_base 7..11: mod_base = OTHER; note = modified with 2'-methoxy
  modified_base 12: mod_base = OTHER; note = modified with 2'-Fluoro
  modified_base 13: mod_base = OTHER; note = modified with 2'-methoxy
  modified_base 14: mod_base = OTHER; note = modified with 2'-Fluoro
  modified_base 15: mod_base = OTHER; note = modified with 2'-methoxy
  modified_base 16: mod_base = OTHER; note = modified with 2'-Fluoro
  modified_base 17..21: mod_base = OTHER; note = modified with 2'-methoxy
  modified_base 1..3: mod_base = OTHER; note = two adjacent nucleosides are linked by phosphorothioate diester groups
  modified_base 19..21: mod_base = OTHER; note = two adjacent nucleosides are linked by phosphorothioate diester groups
  modified_base 1: mod_base = OTHER; note = 5'-E-VP
ttgcagttcagggtagacttc

SEQ ID NO: 127 - RNA, 21 nt, Synthetic Construct
  source 1..21: mol_type = other RNA; note = modified anti-sense strand
  modified_base 1: mod_base = OTHER; note = modified with 2'-methoxy
  modified_base 2: mod_base = OTHER; note = modified with 2'-Fluoro
  modified_base 3..5: mod_base = OTHER; note = modified with 2'-methoxy
  modified_base 6: mod_base = OTHER; note = modified with 2'-Fluoro
  modified_base 7..11: mod_base = OTHER; note = modified with 2'-methoxy
  modified_base 12: mod_base = OTHER; note = modified with 2'-Fluoro
  modified_base 13: mod_base = OTHER; note = modified with 2'-methoxy
  modified_base 14: mod_base = OTHER; note = modified with 2'-Fluoro
  modified_base 15: mod_base = OTHER; note = modified with 2'-methoxy
  modified_base 16: mod_base = OTHER; note = modified with 2'-Fluoro
  modified_base 17..21: mod_base = OTHER; note = modified with 2'-methoxy
  modified_base 1..3: mod_base = OTHER; note = two adjacent nucleosides are linked by phosphorothioate diester groups
  modified_base 19..21: mod_base = OTHER; note = two adjacent nucleosides are linked by phosphorothioate diester groups
  modified_base 1: mod_base = OTHER; note = 5'-E-VP
ttcctcatcgtcctcgtcatc

SEQ ID NO: 128 - RNA, 21 nt, Synthetic Construct
  source 1..21: mol_type = other RNA; note = modified anti-sense strand
  modified_base 1: mod_base = OTHER; note = modified with 2'-methoxy
  modified_base 2: mod_base = OTHER; note = modified with 2'-Fluoro
  modified_base 3..5: mod_base = OTHER; note = modified with 2'-methoxy
  modified_base 6: mod_base = OTHER; note = modified with 2'-Fluoro
  modified_base 7..11: mod_base = OTHER; note = modified with 2'-methoxy
  modified_base 12: mod_base = OTHER; note = modified with 2'-Fluoro
  modified_base 13: mod_base = OTHER; note = modified with 2'-methoxy
  modified_base 14: mod_base = OTHER; note = modified with 2'-Fluoro
  modified_base 15: mod_base = OTHER; note = modified with 2'-methoxy
  modified_base 16: mod_base = OTHER; note = modified with 2'-Fluoro
  modified_base 17..21: mod_base = OTHER; note = modified with 2'-methoxy
  modified_base 1..3: mod_base = OTHER; note = two adjacent nucleosides are linked by phosphorothioate diester groups
  modified_base 19..21: mod_base = OTHER; note = two adjacent nucleosides are linked by phosphorothioate diester groups
  modified_base 1: mod_base = OTHER; note = 5'-E-VP
tagctgaactcccacgttcac

SEQ ID NO: 129 - RNA, 21 nt, Synthetic Construct
  source 1..21: mol_type = other RNA; note = modified anti-sense strand
  modified_base 1: mod_base = OTHER; note = modified with 2'-methoxy
  modified_base 2: mod_base = OTHER; note = modified with 2'-Fluoro
  modified_base 3..5: mod_base = OTHER; note = modified with 2'-methoxy
  modified_base 6: mod_base = OTHER; note = modified with 2'-Fluoro
  modified_base 7..11: mod_base = OTHER; note = modified with 2'-methoxy
  modified_base 12: mod_base = OTHER; note = modified with 2'-Fluoro
  modified_base 13: mod_base = OTHER; note = modified with 2'-methoxy
  modified_base 14: mod_base = OTHER; note = modified with 2'-Fluoro
  modified_base 15: mod_base = OTHER; note = modified with 2'-methoxy
  modified_base 16: mod_base = OTHER; note = modified with 2'-Fluoro
  modified_base 17..21: mod_base = OTHER; note = modified with 2'-methoxy
  modified_base 1..3: mod_base = OTHER; note = two adjacent nucleosides are linked by phosphorothioate diester groups
  modified_base 19..21: mod_base = OTHER; note = two adjacent nucleosides are linked by phosphorothioate diester groups
  modified_base 1: mod_base = OTHER; note = 5'-E-VP
tagcatctgaaatacttaaaa

SEQ ID NO: 130 - RNA, 21 nt, Synthetic Construct
  source 1..21: mol_type = other RNA; note = modified anti-sense strand
  modified_base 1: mod_base = OTHER; note = modified with 2'-methoxy
  modified_base 2: mod_base = OTHER; note = modified with 2'-Fluoro
  modified_base 3..5: mod_base = OTHER; note = modified with 2'-methoxy
  modified_base 6: mod_base = OTHER; note = modified with 2'-Fluoro
  modified_base 7..11: mod_base = OTHER; note = modified with 2'-methoxy
  modified_base 12: mod_base = OTHER; note = modified with 2'-Fluoro
  modified_base 13: mod_base = OTHER; note = modified with 2'-methoxy
  modified_base 14: mod_base = OTHER; note = modified with 2'-Fluoro
  modified_base 15: mod_base = OTHER; note = modified with 2'-methoxy
  modified_base 16: mod_base = OTHER; note = modified with 2'-Fluoro
  modified_base 17..21: mod_base = OTHER; note = modified with 2'-methoxy
  modified_base 1..3: mod_base = OTHER; note = two adjacent nucleosides are linked by phosphorothioate diester groups
  modified_base 19..21: mod_base = OTHER; note = two adjacent nucleosides are linked by phosphorothioate diester groups
  modified_base 1: mod_base = OTHER; note = 5'-E-VP
tagaccagcagagcacccctc

SEQ ID NO: 131 - RNA, 21 nt, Synthetic Construct
  source 1..21: mol_type = other RNA; note = modified anti-sense strand
  modified_base 1: mod_base = OTHER; note = modified with 2'-methoxy
  modified_base 2: mod_base = OTHER; note = modified with 2'-Fluoro
  modified_base 3..5: mod_base = OTHER; note = modified with 2'-methoxy
  modified_base 6: mod_base = OTHER; note = modified with 2'-Fluoro
  modified_base 7..11: mod_base = OTHER; note = modified with 2'-methoxy
  modified_base 12: mod_base = OTHER; note = modified with 2'-Fluoro
  modified_base 13: mod_base = OTHER; note = modified with 2'-methoxy
  modified_base 14: mod_base = OTHER; note = modified with 2'-Fluoro
  modified_base 15: mod_base = OTHER; note = modified with 2'-methoxy
  modified_base 16: mod_base = OTHER; note = modified with 2'-Fluoro
  modified_base 17..21: mod_base = OTHER; note = modified with 2'-methoxy
  modified_base 1..3: mod_base = OTHER; note = two adjacent nucleosides are linked by phosphorothioate diester groups
  modified_base 19..21: mod_base = OTHER; note = two adjacent nucleosides are linked by phosphorothioate diester groups
  modified_base 1: mod_base = OTHER; note = 5'-E-VP
tgaagaccagcagagcacccc

SEQ ID NO: 132 - RNA, 21 nt, Synthetic Construct
  source 1..21: mol_type = other RNA; note = modified anti-sense strand
  modified_base 1: mod_base = OTHER; note = modified with 2'-methoxy
  modified_base 2: mod_base = OTHER; note = modified with 2'-Fluoro
  modified_base 3..5: mod_base = OTHER; note = modified with 2'-methoxy
  modified_base 6: mod_base = OTHER; note = modified with 2'-Fluoro
  modified_base 7..11: mod_base = OTHER; note = modified with 2'-methoxy
  modified_base 12: mod_base = OTHER; note = modified with 2'-Fluoro
  modified_base 13: mod_base = OTHER; note = modified with 2'-methoxy
  modified_base 14: mod_base = OTHER; note = modified with 2'-Fluoro
  modified_base 15: mod_base = OTHER; note = modified with 2'-methoxy
  modified_base 16: mod_base = OTHER; note = modified with 2'-Fluoro
  modified_base 17..21: mod_base = OTHER; note = modified with 2'-methoxy
  modified_base 1..3: mod_base = OTHER; note = two adjacent nucleosides are linked by phosphorothioate diester groups
  modified_base 19..21: mod_base = OTHER; note = two adjacent nucleosides are linked by phosphorothioate diester groups
  modified_base 1: mod_base = OTHER; note = 5'-E-VP
ttgaagaccagcagagcaccc

SEQ ID NO: 133 - RNA, 21 nt, Synthetic Construct
  source 1..21: mol_type = other RNA; note = modified anti-sense strand
  modified_base 1: mod_base = OTHER; note = modified with 2'-methoxy
  modified_base 2: mod_base = OTHER; note = modified with 2'-Fluoro
  modified_base 3: mod_base = OTHER; note = modified with 2'-methoxy
  modified_base 4: mod_base = OTHER; note = modified with 2'-Fluoro
  modified_base 5: mod_base = OTHER; note = modified with 2'-methoxy
  modified_base 6: mod_base = OTHER; note = modified with 2'-Fluoro
  modified_base 7..9: mod_base = OTHER; note = modified with 2'-methoxy
  modified_base 10: mod_base = OTHER; note = modified with 2'-Fluoro
  modified_base 11: mod_base = OTHER; note = modified with 2'-methoxy
  modified_base 12: mod_base = OTHER; note = modified with 2'-Fluoro
  modified_base 13: mod_base = OTHER; note = modified with 2'-methoxy
  modified_base 14: mod_base = OTHER; note = modified with 2'-Fluoro
  modified_base 15: mod_base = OTHER; note = modified with 2'-methoxy
  modified_base 16: mod_base = OTHER; note = modified with 2'-Fluoro
  modified_base 17: mod_base = OTHER; note = modified with 2'-methoxy
  modified_base 18: mod_base = OTHER; note = modified with 2'-Fluoro
  modified_base 19..21: mod_base = OTHER; note = modified with 2'-methoxy
  modified_base 1..3: mod_base = OTHER; note = two adjacent nucleosides are linked by phosphorothioate diester groups
  modified_base 19..21: mod_base = OTHER; note = two adjacent nucleosides are linked by phosphorothioate diester groups
ttgcagttcagggtagacttc

SEQ ID NO: 134 - RNA, 21 nt, Synthetic Construct
  source 1..21: mol_type = other RNA; note = modified anti-sense strand
  modified_base 1: mod_base = OTHER; note = modified with 2'-methoxy
  modified_base 2: mod_base = OTHER; note = modified with 2'-Fluoro
  modified_base 3: mod_base = OTHER; note = modified with 2'-methoxy
  modified_base 4: mod_base = OTHER; note = modified with 2'-Fluoro
  modified_base 5: mod_base = OTHER; note = modified with 2'-methoxy
  modified_base 6: mod_base = OTHER; note = modified with 2'-Fluoro
  modified_base 7..9: mod_base = OTHER; note = modified with 2'-methoxy
  modified_base 10: mod_base = OTHER; note = modified with 2'-Fluoro
  modified_base 11: mod_base = OTHER; note = modified with 2'-methoxy
  modified_base 12: mod_base = OTHER; note = modified with 2'-Fluoro
  modified_base 13: mod_base = OTHER; note = modified with 2'-methoxy
  modified_base 14: mod_base = OTHER; note = modified with 2'-Fluoro
  modified_base 15: mod_base = OTHER; note = modified with 2'-methoxy
  modified_base 16: mod_base = OTHER; note = modified with 2'-Fluoro
  modified_base 17: mod_base = OTHER; note = modified with 2'-methoxy
  modified_base 18: mod_base = OTHER; note = modified with 2'-Fluoro
  modified_base 19..21: mod_base = OTHER; note = modified with 2'-methoxy
  modified_base 1..3: mod_base = OTHER; note = two adjacent nucleosides are linked by phosphorothioate diester groups
  modified_base 19..21: mod_base = OTHER; note = two adjacent nucleosides are linked by phosphorothioate diester groups
ttcctcatcgtcctcgtcatc

SEQ ID NO: 135 - RNA, 21 nt, Synthetic Construct
  source 1..21: mol_type = other RNA; note = modified anti-sense strand
  modified_base 1: mod_base = OTHER; note = modified with 2'-methoxy
  modified_base 2: mod_base = OTHER; note = modified with 2'-Fluoro
  modified_base 3: mod_base = OTHER; note = modified with 2'-methoxy
  modified_base 4: mod_base = OTHER; note = modified with 2'-Fluoro
  modified_base 5: mod_base = OTHER; note = modified with 2'-methoxy
  modified_base 6: mod_base = OTHER; note = modified with 2'-Fluoro
  modified_base 7..9: mod_base = OTHER; note = modified with 2'-methoxy
  modified_base 10: mod_base = OTHER; note = modified with 2'-Fluoro
  modified_base 11: mod_base = OTHER; note = modified with 2'-methoxy
  modified_base 12: mod_base = OTHER; note = modified with 2'-Fluoro
  modified_base 13: mod_base = OTHER; note = modified with 2'-methoxy
  modified_base 14: mod_base = OTHER; note = modified with 2'-Fluoro
  modified_base 15: mod_base = OTHER; note = modified with 2'-methoxy
  modified_base 16: mod_base = OTHER; note = modified with 2'-Fluoro
  modified_base 17: mod_base = OTHER; note = modified with 2'-methoxy
  modified_base 18: mod_base = OTHER; note = modified with 2'-Fluoro
  modified_base 19..21: mod_base = OTHER; note = modified with 2'-methoxy
  modified_base 1..3: mod_base = OTHER; note = two adjacent nucleosides are linked by phosphorothioate diester groups
  modified_base 19..21: mod_base = OTHER; note = two adjacent nucleosides are linked by phosphorothioate diester groups
tagctgaactcccacgttcac

SEQ ID NO: 136 - RNA, 21 nt, Synthetic Construct
  source 1..21: mol_type = other RNA; note = modified anti-sense strand
  modified_base 1: mod_base = OTHER; note = modified with 2'-methoxy
  modified_base 2: mod_base = OTHER; note = modified with 2'-Fluoro
  modified_base 3: mod_base = OTHER; note = modified with 2'-methoxy
  modified_base 4: mod_base = OTHER; note = modified with 2'-Fluoro
  modified_base 5: mod_base = OTHER; note = modified with 2'-methoxy
  modified_base 6: mod_base = OTHER; note = modified with 2'-Fluoro
  modified_base 7..9: mod_base = OTHER; note = modified with 2'-methoxy
  modified_base 10: mod_base = OTHER; note = modified with 2'-Fluoro
  modified_base 11: mod_base = OTHER; note = modified with 2'-methoxy
  modified_base 12: mod_base = OTHER; note = modified with 2'-Fluoro
  modified_base 13: mod_base = OTHER; note = modified with 2'-methoxy
  modified_base 14: mod_base = OTHER; note = modified with 2'-Fluoro
  modified_base 15: mod_base = OTHER; note = modified with 2'-methoxy
  modified_base 16: mod_base = OTHER; note = modified with 2'-Fluoro
  modified_base 17: mod_base = OTHER; note = modified with 2'-methoxy
  modified_base 18: mod_base = OTHER; note = modified with 2'-Fluoro
  modified_base 19..21: mod_base = OTHER; note = modified with 2'-methoxy
  modified_base 1..3: mod_base = OTHER; note = two adjacent nucleosides are linked by phosphorothioate diester groups
  modified_base 19..21: mod_base = OTHER; note = two adjacent nucleosides are linked by phosphorothioate diester groups
tagcatctgaaatacttaaaa

SEQ ID NO: 137 - RNA, 21 nt, Synthetic Construct
  source 1..21: mol_type = other RNA; note = modified anti-sense strand
  modified_base 1: mod_base = OTHER; note = modified with 2'-methoxy
  modified_base 2: mod_base = OTHER; note = modified with 2'-Fluoro
  modified_base 3: mod_base = OTHER; note = modified with 2'-methoxy
  modified_base 4: mod_base = OTHER; note = modified with 2'-Fluoro
  modified_base 5: mod_base = OTHER; note = modified with 2'-methoxy
  modified_base 6: mod_base = OTHER; note = modified with 2'-Fluoro
  modified_base 7..9: mod_base = OTHER; note = modified with 2'-methoxy
  modified_base 10: mod_base = OTHER; note = modified with 2'-Fluoro
  modified_base 11: mod_base = OTHER; note = modified with 2'-methoxy
  modified_base 12: mod_base = OTHER; note = modified with 2'-Fluoro
  modified_base 13: mod_base = OTHER; note = modified with 2'-methoxy
  modified_base 14: mod_base = OTHER; note = modified with 2'-Fluoro
  modified_base 15: mod_base = OTHER; note = modified with 2'-methoxy
  modified_base 16: mod_base = OTHER; note = modified with 2'-Fluoro
  modified_base 17: mod_base = OTHER; note = modified with 2'-methoxy
  modified_base 18: mod_base = OTHER; note = modified with 2'-Fluoro
  modified_base 19..21: mod_base = OTHER; note = modified with 2'-methoxy
  modified_base 1..3: mod_base = OTHER; note = two adjacent nucleosides are linked by phosphorothioate diester groups
  modified_base 19..21: mod_base = OTHER; note = two adjacent nucleosides are linked by phosphorothioate diester groups
tagaccagcagagcacccctc

SEQ ID NO: 138 - RNA, 21 nt, Synthetic Construct
  source 1..21: mol_type = other RNA; note = modified anti-sense strand
  modified_base 1: mod_base = OTHER; note = modified with 2'-methoxy
  modified_base 2: mod_base = OTHER; note = modified with 2'-Fluoro
  modified_base 3: mod_base = OTHER; note = modified with 2'-methoxy
  modified_base 4: mod_base = OTHER; note = modified with 2'-Fluoro
  modified_base 5: mod_base = OTHER; note = modified with 2'-methoxy
  modified_base 6: mod_base = OTHER; note = modified with 2'-Fluoro
  modified_base 7..9: mod_base = OTHER; note = modified with 2'-methoxy
  modified_base 10: mod_base = OTHER; note = modified with 2'-Fluoro
  modified_base 11: mod_base = OTHER; note = modified with 2'-methoxy
  modified_base 12: mod_base = OTHER; note = modified with 2'-Fluoro
  modified_base 13: mod_base = OTHER; note = modified with 2'-methoxy
  modified_base 14: mod_base = OTHER; note = modified with 2'-Fluoro
  modified_base 15: mod_base = OTHER; note = modified with 2'-methoxy
  modified_base 16: mod_base = OTHER; note = modified with 2'-Fluoro
  modified_base 17: mod_base = OTHER; note = modified with 2'-methoxy
  modified_base 18: mod_base = OTHER; note = modified with 2'-Fluoro
  modified_base 19..21: mod_base = OTHER; note = modified with 2'-methoxy
  modified_base 1..3: mod_base = OTHER; note = two adjacent nucleosides are linked by phosphorothioate diester groups
  modified_base 19..21: mod_base = OTHER; note = two adjacent nucleosides are linked by phosphorothioate diester groups
tgaagaccagcagagcacccc

SEQ ID NO: 139 - RNA, 21 nt, Synthetic Construct
  source 1..21: mol_type = other RNA; note = modified anti-sense strand
  modified_base 1: mod_base = OTHER; note = modified with 2'-methoxy
  modified_base 2: mod_base = OTHER; note = modified with 2'-Fluoro
  modified_base 3: mod_base = OTHER; note = modified with 2'-methoxy
  modified_base 4: mod_base = OTHER; note = modified with 2'-Fluoro
  modified_base 5: mod_base = OTHER; note = modified with 2'-methoxy
  modified_base 6: mod_base = OTHER; note = modified with 2'-Fluoro
  modified_base 7..9: mod_base = OTHER; note = modified with 2'-methoxy
  modified_base 10: mod_base = OTHER; note = modified with 2'-Fluoro
  modified_base 11: mod_base = OTHER; note = modified with 2'-methoxy
  modified_base 12: mod_base = OTHER; note = modified with 2'-Fluoro
  modified_base 13: mod_base = OTHER; note = modified with 2'-methoxy
  modified_base 14: mod_base = OTHER; note = modified with 2'-Fluoro
  modified_base 15: mod_base = OTHER; note = modified with 2'-methoxy
  modified_base 16: mod_base = OTHER; note = modified with 2'-Fluoro
  modified_base 17: mod_base = OTHER; note = modified with 2'-methoxy
  modified_base 18: mod_base = OTHER; note = modified with 2'-Fluoro
  modified_base 19..21: mod_base = OTHER; note = modified with 2'-methoxy
  modified_base 1..3: mod_base = OTHER; note = two adjacent nucleosides are linked by phosphorothioate diester groups
  modified_base 19..21: mod_base = OTHER; note = two adjacent nucleosides are linked by phosphorothioate diester groups
ttgaagaccagcagagcaccc

SEQ ID NO: 140 - RNA, 21 nt, Synthetic Construct
  source 1..21: mol_type = other RNA; note = modified anti-sense strand
  modified_base 1: mod_base = OTHER; note = modified with 2'-methoxy
  modified_base 2: mod_base = OTHER; note = modified with 2'-Fluoro
  modified_base 3..5: mod_base = OTHER; note = modified with 2'-methoxy
  modified_base 6: mod_base = OTHER; note = modified with 2'-Fluoro
  modified_base 7..11: mod_base = OTHER; note = modified with 2'-methoxy
  modified_base 12: mod_base = OTHER; note = modified with 2'-Fluoro
  modified_base 13: mod_base = OTHER; note = modified with 2'-methoxy
  modified_base 14: mod_base = OTHER; note = modified with 2'-Fluoro
  modified_base 15: mod_base = OTHER; note = modified with 2'-methoxy
  modified_base 16: mod_base = OTHER; note = modified with 2'-Fluoro
  modified_base 17..21: mod_base = OTHER; note = modified with 2'-methoxy
  modified_base 1..3: mod_base = OTHER; note = two adjacent nucleosides are linked by phosphorothioate diester groups
  modified_base 19..21: mod_base = OTHER; note = two adjacent nucleosides are linked by phosphorothioate diester groups
  modified_base 1: mod_base = OTHER; note = 5'-E-VP
tagcatctgaaatacttaaaa

SEQ ID NO: 141 - RNA, 21 nt, Synthetic Construct
  source 1..21: mol_type = other RNA; note = modified anti-sense strand
  modified_base 1: mod_base = OTHER; note = modified with 2'-methoxy
  modified_base 2: mod_base = OTHER; note = modified with 2'-Fluoro
  modified_base 3..5: mod_base = OTHER; note = modified with 2'-methoxy
  modified_base 6: mod_base = OTHER; note = modified with 2'-Fluoro
  modified_base 7..11: mod_base = OTHER; note = modified with 2'-methoxy
  modified_base 12: mod_base = OTHER; note = modified with 2'-Fluoro
  modified_base 13: mod_base = OTHER; note = modified with 2'-methoxy
  modified_base 14: mod_base = OTHER; note = modified with 2'-Fluoro
  modified_base 15: mod_base = OTHER; note = modified with 2'-methoxy
  modified_base 16: mod_base = OTHER; note = modified with 2'-Fluoro
  modified_base 17..21: mod_base = OTHER; note = modified with 2'-methoxy
  modified_base 1..3: mod_base = OTHER; note = two adjacent nucleosides are linked by phosphorothioate diester groups
  modified_base 19..21: mod_base = OTHER; note = two adjacent nucleosides are linked by phosphorothioate diester groups
  modified_base 1: mod_base = OTHER; note = 5'-E-VP
tagcatctgaaatacttaaaa

SEQ ID NO: 142 - RNA, 21 nt, Synthetic Construct
  source 1..21: mol_type = other RNA; note = modified anti-sense strand
  modified_base 1: mod_base = OTHER; note = modified with 2'-methoxy
  modified_base 2: mod_base = OTHER; note = modified with 2'-Fluoro
  modified_base 3..5: mod_base = OTHER; note = modified with 2'-methoxy
  modified_base 6: mod_base = OTHER; note = modified with 2'-Fluoro
  modified_base 7..11: mod_base = OTHER; note = modified with 2'-methoxy
  modified_base 12: mod_base = OTHER; note = modified with 2'-Fluoro
  modified_base 13: mod_base = OTHER; note = modified with 2'-methoxy
  modified_base 14: mod_base = OTHER; note = modified with 2'-Fluoro
  modified_base 15: mod_base = OTHER; note = modified with 2'-methoxy
  modified_base 16: mod_base = OTHER; note = modified with 2'-Fluoro
  modified_base 17..21: mod_base = OTHER; note = modified with 2'-methoxy
  modified_base 1..3: mod_base = OTHER; note = two adjacent nucleosides are linked by phosphorothioate diester groups
  modified_base 19..21: mod_base = OTHER; note = two adjacent nucleosides are linked by phosphorothioate diester groups
  modified_base 1: mod_base = OTHER; note = 5'-E-VP
tagcatctgaaatacttaaaa

SEQ ID NO: 143 - RNA, 19 nt, Synthetic Construct
  source 1..19: mol_type = other RNA; note = modified sense strand
  modified_base 1..6: mod_base = OTHER; note = modified with 2'-methoxy
  modified_base 7..9: mod_base = OTHER; note = modified with 2'-Fluoro
  modified_base 10..19: mod_base = OTHER; note = modified with 2'-methoxy
  modified_base 1..3: mod_base = OTHER; note = two adjacent nucleosides are linked by phosphorothioate diester groups
cgaggacgatgaggatgga

SEQ ID NO: 144 - RNA, 19 nt, Synthetic Construct
  source 1..19: mol_type = other RNA; note = modified sense strand
  modified_base 1..6: mod_base = OTHER; note = modified with 2'-methoxy
  modified_base 7..9: mod_base = OTHER; note = modified with 2'-Fluoro
  modified_base 10..19: mod_base = OTHER; note = modified with 2'-methoxy
  modified_base 1..3: mod_base = OTHER; note = two adjacent nucleosides are linked by phosphorothioate diester groups
ggacgatgaggatggtgaa

SEQ ID NO: 145 - RNA, 19 nt, Synthetic Construct
  source 1..19: mol_type = other RNA; note = modified sense strand
  modified_base 1..6: mod_base = OTHER; note = modified with 2'-methoxy
  modified_base 7..9: mod_base = OTHER; note = modified with 2'-Fluoro
  modified_base 10..19: mod_base = OTHER; note = modified with 2'-methoxy
  modified_base 1..3: mod_base = OTHER; note = two adjacent nucleosides are linked by phosphorothioate diester groups
cgatgaggatggtgatgaa

SEQ ID NO: 146 - RNA, 19 nt, Synthetic Construct
  source 1..19: mol_type = other RNA; note = modified sense strand
  modified_base 1..6: mod_base = OTHER; note = modified with 2'-methoxy
  modified_base 7..9: mod_base = OTHER; note = modified with 2'-Fluoro
  modified_base 10..19: mod_base = OTHER; note = modified with 2'-methoxy
  modified_base 1..3: mod_base = OTHER; note = two adjacent nucleosides are linked by phosphorothioate diester groups
ggctgaggaaccctacgaa

SEQ ID NO: 147 - RNA, 19 nt, Synthetic Construct
  source 1..19: mol_type = other RNA; note = modified sense strand
  modified_base 1..6: mod_base = OTHER; note = modified with 2'-methoxy
  modified_base 7..9: mod_base = OTHER; note = modified with 2'-Fluoro
  modified_base 10..19: mod_base = OTHER; note = modified with 2'-methoxy
  modified_base 1..3: mod_base = OTHER; note = two adjacent nucleosides are linked by phosphorothioate diester groups
gctgaggaaccctacgaaa

SEQ ID NO: 148 - RNA, 19 nt, Synthetic Construct
  source 1..19: mol_type = other RNA; note = modified sense strand
  modified_base 1..6: mod_base = OTHER; note = modified with 2'-methoxy
  modified_base 7..9: mod_base = OTHER; note = modified with 2'-Fluoro
  modified_base 10..19: mod_base = OTHER; note = modified with 2'-methoxy
  modified_base 1..3: mod_base = OTHER; note = two adjacent nucleosides are linked by phosphorothioate diester groups
ctgaggaaccctacgaaga

SEQ ID NO: 149 - RNA, 19 nt, Synthetic Construct
  source 1..19: mol_type = other RNA; note = modified sense strand
  modified_base 1..6: mod_base = OTHER; note = modified with 2'-methoxy
  modified_base 7..9: mod_base = OTHER; note = modified with 2'-Fluoro
  modified_base 10..19: mod_base = OTHER; note = modified with 2'-methoxy
  modified_base 1..3: mod_base = OTHER; note = two adjacent nucleosides are linked by phosphorothioate diester groups
tgaggaaccctacgaagaa

SEQ ID NO: 150 - RNA, 19 nt, Synthetic Construct
  source 1..19: mol_type = other RNA; note = modified sense strand
  modified_base 1..6: mod_base = OTHER; note = modified with 2'-methoxy
  modified_base 7..9: mod_base = OTHER; note = modified with 2'-Fluoro
  modified_base 10..19: mod_base = OTHER; note = modified with 2'-methoxy
  modified_base 1..3: mod_base = OTHER; note = two adjacent nucleosides are linked by phosphorothioate diester groups
gaggaaccctacgaagaaa

SEQ ID NO: 151 - RNA, 19 nt, Synthetic Construct
  source 1..19: mol_type = other RNA; note = modified sense strand
  modified_base 1..6: mod_base = OTHER; note = modified with 2'-methoxy
  modified_base 7..9: mod_base = OTHER; note = modified with 2'-Fluoro
  modified_base 10..19: mod_base = OTHER; note = modified with 2'-methoxy
  modified_base 1..3: mod_base = OTHER; note = two adjacent nucleosides are linked by phosphorothioate diester groups
gaaccctacgaagaagcca

SEQ ID NO: 152 - RNA, 19 nt, Synthetic Construct
  source 1..19: mol_type = other RNA; note = modified sense strand
  modified_base 1..6: mod_base = OTHER; note = modified with 2'-methoxy
  modified_base 7..9: mod_base = OTHER; note = modified with 2'-Fluoro
  modified_base 10..19: mod_base = OTHER; note = modified with 2'-methoxy
  modified_base 1..3: mod_base = OTHER; note = two adjacent nucleosides are linked by phosphorothioate diester groups
accctacgaagaagccaca

SEQ ID NO: 153 - RNA, 19 nt, Synthetic Construct
  source 1..19: mol_type = other RNA; note = modified sense strand
  modified_base 1..6: mod_base = OTHER; note = modified with 2'-methoxy
  modified_base 7..9: mod_base = OTHER; note = modified with 2'-Fluoro
  modified_base 10..19: mod_base = OTHER; note = modified with 2'-methoxy
  modified_base 1..3: mod_base = OTHER; note = two adjacent nucleosides are linked by phosphorothioate diester groups
cctacgaagaagccacaga

SEQ ID NO: 154 - RNA, 19 nt, Synthetic Construct
  source 1..19: mol_type = other RNA; note = modified sense strand
  modified_base 1..6: mod_base = OTHER; note = modified with 2'-methoxy
  modified_base 7..9: mod_base = OTHER; note = modified with 2'-Fluoro
  modified_base 10..19: mod_base = OTHER; note = modified with 2'-methoxy
  modified_base 1..3: mod_base = OTHER; note = two adjacent nucleosides are linked by phosphorothioate diester groups
tacgaagaagccacagaga

SEQ ID NO: 155 - RNA, 19 nt, Synthetic Construct
  source 1..19: mol_type = other RNA; note = modified sense strand
  modified_base 1..6: mod_base = OTHER; note = modified with 2'-methoxy
  modified_base 7..9: mod_base = OTHER; note = modified with 2'-Fluoro
  modified_base 10..19: mod_base = OTHER; note = modified with 2'-methoxy
  modified_base 1..3: mod_base = OTHER; note = two adjacent nucleosides are linked by phosphorothioate diester groups
cgaagaagccacagagaga

SEQ ID NO: 156 - RNA, 19 nt, Synthetic Construct
  source 1..19: mol_type = other RNA; note = modified sense strand
  modified_base 1..6: mod_base = OTHER; note = modified with 2'-methoxy
  modified_base 7..9: mod_base = OTHER; note = modified with 2'-Fluoro
  modified_base 10..19: mod_base = OTHER; note = modified with 2'-methoxy
  modified_base 1..3: mod_base = OTHER; note = two adjacent nucleosides are linked by phosphorothioate diester groups
gaagaagccacagagagaa

SEQ ID NO: 157 - RNA, 19 nt, Synthetic Construct
  source 1..19: mol_type = other RNA; note = modified sense strand
  modified_base 1..6: mod_base = OTHER; note = modified with 2'-methoxy
  modified_base 7..9: mod_base = OTHER; note = modified with 2'-Fluoro
  modified_base 10..19: mod_base = OTHER; note = modified with 2'-methoxy
  modified_base 1..3: mod_base = OTHER; note = two adjacent nucleosides are linked by phosphorothioate diester groups
gaagccacagagagaacca

SEQ ID NO: 158 - RNA, 19 nt, Synthetic Construct
  source 1..19: mol_type = other RNA; note = modified sense strand
  modified_base 1..6: mod_base = OTHER; note = modified with 2'-methoxy
  modified_base 7..9: mod_base = OTHER; note = modified with 2'-Fluoro
  modified_base 10..19: mod_base = OTHER; note = modified with 2'-methoxy
  modified_base 1..3: mod_base = OTHER; note = two adjacent nucleosides are linked by phosphorothioate diester groups
gccacagagagaaccacca

SEQ ID NO: 159 - RNA, 19 nt, Synthetic Construct
  source 1..19: mol_type = other RNA; note = modified sense strand
  modified_base 1..6: mod_base = OTHER; note = modified with 2'-methoxy
  modified_base 7..9: mod_base = OTHER; note = modified with 2'-Fluoro
  modified_base 10..19: mod_base = OTHER; note = modified with 2'-methoxy
  modified_base 1..3: mod_base = OTHER; note = two adjacent nucleosides are linked by phosphorothioate diester groups
ccacagagagaaccaccaa

SEQ ID NO: 160 - RNA, 19 nt, Synthetic Construct
  source 1..19: mol_type = other RNA; note = modified sense strand
  modified_base 1..6: mod_base = OTHER; note = modified with 2'-methoxy
  modified_base 7..9: mod_base = OTHER; note = modified with 2'-Fluoro
  modified_base 10..19: mod_base = OTHER; note = modified with 2'-methoxy
  modified_base 1..3: mod_base = OTHER; note = two adjacent nucleosides are linked by phosphorothioate diester groups
gccaccaccaccaccacca

SEQ ID NO: 161 - RNA, 19 nt, Synthetic Construct
  source 1..19: mol_type = other RNA; note = modified sense strand
  modified_base 1..6: mod_base = OTHER; note = modified with 2'-methoxy
  modified_base 7..9: mod_base = OTHER; note = modified with 2'-Fluoro
  modified_base 10..19: mod_base = OTHER; note = modified with 2'-methoxy
  modified_base 1..3: mod_base = OTHER; note = two adjacent nucleosides are linked by phosphorothioate diester groups
gagaggtgtgctctgaaca

SEQ ID NO: 162 - RNA, 19 nt, Synthetic Construct
  source 1..19: mol_type = other RNA; note = modified sense strand
  modified_base 1..6: mod_base = OTHER; note = modified with 2'-methoxy
  modified_base 7..9: mod_base = OTHER; note = modified with 2'-Fluoro
  modified_base 10..19: mod_base = OTHER; note = modified with 2'-methoxy
  modified_base 1..3: mod_base = OTHER; note = two adjacent nucleosides are linked by phosphorothioate diester groups
agaggtgtgctctgaacaa

SEQ ID NO: 163 - RNA, 19 nt, Synthetic Construct
  source 1..19: mol_type = other RNA; note = modified sense strand
  modified_base 1..6: mod_base = OTHER; note = modified with 2'-methoxy
  modified_base 7..9: mod_base = OTHER; note = modified with 2'-Fluoro
  modified_base 10..19: mod_base = OTHER; note = modified with 2'-methoxy
  modified_base 1..3: mod_base = OTHER; note = two adjacent nucleosides are linked by phosphorothioate diester groups
ggccgtgccgagcaatgaa

SEQ ID NO: 164 - RNA, 19 nt, Synthetic Construct
  source 1..19: mol_type = other RNA; note = modified sense strand
  modified_base 1..6: mod_base = OTHER; note = modified with 2'-methoxy
  modified_base 7..9: mod_base = OTHER; note = modified with 2'-Fluoro
  modified_base 10..19: mod_base = OTHER; note = modified with 2'-methoxy
  modified_base 1..3: mod_base = OTHER; note = two adjacent nucleosides are linked by phosphorothioate diester groups
ccgtgccgagcaatgatca

SEQ ID NO: 165 - RNA, 19 nt, Synthetic Construct
  source 1..19: mol_type = other RNA; note = modified sense strand
  modified_base 1..6: mod_base = OTHER; note = modified with 2'-methoxy
  modified_base 7..9: mod_base = OTHER; note = modified with 2'-Fluoro
  modified_base 10..19: mod_base = OTHER; note = modified with 2'-methoxy
  modified_base 1..3: mod_base = OTHER; note = two adjacent nucleosides are linked by phosphorothioate diester groups
cgtgccgagcaatgatcta

SEQ ID NO: 166 - RNA, 19 nt, Synthetic Construct
  source 1..19: mol_type = other RNA; note = modified sense strand
  modified_base 1..6: mod_base = OTHER; note = modified with 2'-methoxy
  modified_base 7..9: mod_base = OTHER; note = modified with 2'-Fluoro
  modified_base 10..19: mod_base = OTHER; note = modified with 2'-methoxy
  modified_base 1..3: mod_base = OTHER; note = two adjacent nucleosides are linked by phosphorothioate diester groups
ggatgtggcggcaaccgga

SEQ ID NO: 167 - RNA, 19 nt, Synthetic Construct
  source 1..19: mol_type = other RNA; note = modified sense strand
  modified_base 1..6: mod_base = OTHER; note = modified with 2'-methoxy
  modified_base 7..9: mod_base = OTHER; note = modified with 2'-Fluoro
  modified_base 10..19: mod_base = OTHER; note = modified with 2'-methoxy
  modified_base 1..3: mod_base = OTHER; note = two adjacent nucleosides are linked by phosphorothioate diester groups
gatgtggcggcaaccggaa

SEQ ID NO: 168 - RNA, 19 nt, Synthetic Construct
  source 1..19: mol_type = other RNA; note = modified sense strand
  modified_base 1..6: mod_base = OTHER; note = modified with 2'-methoxy
  modified_base 7..9: mod_base = OTHER; note = modified with 2'-Fluoro
  modified_base 10..19: mod_base = OTHER; note = modified with 2'-methoxy
  modified_base 1..3: mod_base = OTHER; note = two adjacent nucleosides are linked by phosphorothioate diester groups
ggcggcaaccggaacaaca

SEQ ID NO: 169 - RNA, 19 nt, Synthetic Construct
  source 1..19: mol_type = other RNA; note = modified sense strand
  modified_base 1..6: mod_base = OTHER; note = modified with 2'-methoxy
  modified_base 7..9: mod_base = OTHER; note = modified with 2'-Fluoro
  modified_base 10..19: mod_base = OTHER; note = modified with 2'-methoxy
  modified_base 1..3: mod_base = OTHER; note = two adjacent nucleosides are linked by phosphorothioate diester groups
gcggcaaccggaacaacta

SEQ ID NO: 170 - RNA, 19 nt, Synthetic Construct
  source 1..19: mol_type = other RNA; note = modified sense strand
  modified_base 1..6: mod_base = OTHER; note = modified with 2'-methoxy
  modified_base 7..9: mod_base = OTHER; note = modified with 2'-Fluoro
  modified_base 10..19: mod_base = OTHER; note = modified with 2'-methoxy
  modified_base 1..3: mod_base = OTHER; note = two adjacent nucleosides are linked by phosphorothioate diester groups
cggcaaccggaacaactta

SEQ ID NO: 171 - RNA, 19 nt, Synthetic Construct
  source 1..19: mol_type = other RNA; note = modified sense strand
  modified_base 1..6: mod_base = OTHER; note = modified with 2'-methoxy
  modified_base 7..9: mod_base = OTHER; note = modified with 2'-Fluoro
  modified_base 10..19: mod_base = OTHER; note = modified with 2'-methoxy
  modified_base 1..3: mod_base = OTHER; note = two adjacent nucleosides are linked by phosphorothioate diester groups
ggcaaccggaacaacttta

SEQ ID NO: 172 - RNA, 19 nt, Synthetic Construct
  source 1..19: mol_type = other RNA; note = modified sense strand
  modified_base 1..6: mod_base = OTHER; note = modified with 2'-methoxy
  modified_base 7..9: mod_base = OTHER; note = modified with 2'-Fluoro
  modified_base 10..19: mod_base = OTHER; note = modified with 2'-methoxy
  modified_base 1..3: mod_base = OTHER; note = two adjacent nucleosides are linked by phosphorothioate diester groups
gcaaccggaacaactttga

SEQ ID NO: 173 - RNA, 19 nt, Synthetic Construct
  source 1..19: mol_type = other RNA; note = modified sense strand
  modified_base 1..6: mod_base = OTHER; note = modified with 2'-methoxy
  modified_base 7..9: mod_base = OTHER; note = modified with 2'-Fluoro
  modified_base 10..19: mod_base = OTHER; note = modified with 2'-methoxy
  modified_base 1..3: mod_base = OTHER; note = two adjacent nucleosides are linked by phosphorothioate diester groups
agaacgtcaagcaaagaaa

SEQ ID NO: 174 - RNA, 19 nt, Synthetic Construct
  source 1..19: mol_type = other RNA; note = modified sense strand
  modified_base 1..6: mod_base = OTHER; note = modified with 2'-methoxy
  modified_base 7..9: mod_base = OTHER; note = modified with 2'-Fluoro
  modified_base 10..19: mod_base = OTHER; note = modified with 2'-methoxy
  modified_base 1..3: mod_base = OTHER; note = two adjacent nucleosides are linked by phosphorothioate diester groups
ggccagagtggaagccata

SEQ ID NO: 175 - RNA, 19 nt, Synthetic Construct
  source 1..19: mol_type = other RNA; note = modified sense strand
  modified_base 1..6: mod_base = OTHER; note = modified with 2'-methoxy
  modified_base 7..9: mod_base = OTHER; note = modified with 2'-Fluoro
  modified_base 10..19: mod_base = OTHER; note = modified with 2'-methoxy
  modified_base 1..3: mod_base = OTHER; note = two adjacent nucleosides are linked by phosphorothioate diester groups
agaacagaaggacagacaa

SEQ ID NO: 176 - RNA, 19 nt, Synthetic Construct
  source 1..19: mol_type = other RNA; note = modified sense strand
  modified_base 1..6: mod_base = OTHER; note = modified with 2'-methoxy
  modified_base 7..9: mod_base = OTHER; note = modified with 2'-Fluoro
  modified_base 10..19: mod_base = OTHER; note = modified with 2'-methoxy
  modified_base 1..3: mod_base = OTHER; note = two adjacent nucleosides are linked by phosphorothioate diester groups
tcacatagccccttagcca

SEQ ID NO: 177 - RNA, 19 nt, Synthetic Construct
  source 1..19: mol_type = other RNA; note = modified sense strand
  modified_base 1..6: mod_base = OTHER; note = modified with 2'-methoxy
  modified_base 7..9: mod_base = OTHER; note = modified with 2'-Fluoro
  modified_base 10..19: mod_base = OTHER; note = modified with 2'-methoxy
  modified_base 1..3: mod_base = OTHER; note = two adjacent nucleosides are linked by phosphorothioate diester groups
gccccttagccagttgtaa

SEQ ID NO: 178 - RNA, 19 nt, Synthetic Construct
  source 1..19: mol_type = other RNA; note = modified sense strand
  modified_base 1..6: mod_base = OTHER; note = modified with 2'-methoxy
  modified_base 7..9: mod_base = OTHER; note = modified with 2'-Fluoro
  modified_base 10..19: mod_base = OTHER; note = modified with 2'-methoxy
  modified_base 1..3: mod_base = OTHER; note = two adjacent nucleosides are linked by phosphorothioate diester groups
ccccttagccagttgtata

SEQ ID NO: 179 - RNA, 19 nt, Synthetic Construct
  source 1..19: mol_type = other RNA; note = modified sense strand
  modified_base 1..6: mod_base = OTHER; note = modified with 2'-methoxy
  modified_base 7..9: mod_base = OTHER; note = modified with 2'-Fluoro
  modified_base 10..19: mod_base = OTHER; note = modified with 2'-methoxy
  modified_base 1..3: mod_base = OTHER; note = two adjacent nucleosides are linked by phosphorothioate diester groups
atgtgaacgtgggagttca

SEQ ID NO: 180 - RNA, 19 nt, Synthetic Construct
  source 1..19: mol_type = other RNA; note = modified sense strand
  modified_base 1..6: mod_base = OTHER; note = modified with 2'-methoxy
  modified_base 7..9: mod_base = OTHER; note = modified with 2'-Fluoro
  modified_base 10..19: mod_base = OTHER; note = modified with 2'-methoxy
  modified_base 1..3: mod_base = OTHER; note = two adjacent nucleosides are linked by phosphorothioate diester groups
taagtatttcagatgctta

SEQ ID NO: 181 - RNA, 19 nt, Synthetic Construct
  source 1..19: mol_type = other RNA; note = modified sense strand
  modified_base 1..6: mod_base = OTHER; note = modified with 2'-methoxy
  modified_base 7..9: mod_base = OTHER; note = modified with 2'-Fluoro
  modified_base 10..19: mod_base = OTHER; note = modified with 2'-methoxy
  modified_base 1..3: mod_base = OTHER; note = two adjacent nucleosides are linked by phosphorothioate diester groups
ggaattaagaggatacaca

SEQ ID NO: 182 - RNA, 19 nt, Synthetic Construct
  source 1..19: mol_type = other RNA; note = modified sense strand
  modified_base 1..6: mod_base = OTHER; note = modified with 2'-methoxy
  modified_base 7..9: mod_base = OTHER; note = modified with 2'-Fluoro
  modified_base 10..19: mod_base = OTHER; note = modified with 2'-methoxy
  modified_base 1..3: mod_base = OTHER; note = two adjacent nucleosides are linked by phosphorothioate diester groups
gaattaagaggatacacaa

SEQ ID NO: 183 - RNA, 19 nt, Synthetic Construct
  source 1..19: mol_type = other RNA; note = modified sense strand
  modified_base 1..6: mod_base = OTHER; note = modified with 2'-methoxy
  modified_base 7..9: mod_base = OTHER; note = modified with 2'-Fluoro
  modified_base 10..19: mod_base = OTHER; note = modified with 2'-methoxy
  modified_base 1..3: mod_base = OTHER; note = two adjacent nucleosides are linked by phosphorothioate diester groups
gcattgagacttcaagcta

SEQ ID NO: 184 - RNA, 19 nt, Synthetic Construct
  source 1..19: mol_type = other RNA; note = modified sense strand
  modified_base 1..6: mod_base = OTHER; note = modified with 2'-methoxy
  modified_base 7..9: mod_base = OTHER; note = modified with 2'-Fluoro
  modified_base 10..19: mod_base = OTHER; note = modified with 2'-methoxy
  modified_base 1..3: mod_base = OTHER; note = two adjacent nucleosides are linked by phosphorothioate diester groups
cattgagacttcaagctta

SEQ ID NO: 185 - RNA, 19 nt, Synthetic Construct
  source 1..19: mol_type = other RNA; note = modified sense strand
  modified_base 1..6: mod_base = OTHER; note = modified with 2'-methoxy
  modified_base 7..9: mod_base = OTHER; note = modified with 2'-Fluoro
  modified_base 10..19: mod_base = OTHER; note = modified with 2'-methoxy
  modified_base 1..3: mod_base = OTHER; note = two adjacent nucleosides are linked by phosphorothioate diester groups
ggaggggtgctctgctgga

SEQ ID NO: 186 - RNA, 21 nt, Synthetic Construct
  source 1..21: mol_type = other RNA; note = modified anti-sense strand
  modified_base 1: mod_base = OTHER; note = modified with 2'-methoxy
  modified_base 2: mod_base = OTHER; note = modified with 2'-Fluoro
  modified_base 3..5: mod_base = OTHER; note = modified with 2'-methoxy
  modified_base 6: mod_base = OTHER; note = modified with 2'-Fluoro
  modified_base 7..11: mod_base = OTHER; note = modified with 2'-methoxy
  modified_base 12: mod_base = OTHER; note = modified with 2'-Fluoro
  modified_base 13: mod_base = OTHER; note = modified with 2'-methoxy
  modified_base 14: mod_base = OTHER; note = modified with 2'-Fluoro
  modified_base 15: mod_base = OTHER; note = modified with 2'-methoxy
  modified_base 16: mod_base = OTHER; note = modified with 2'-Fluoro
  modified_base 17..21: mod_base = OTHER; note = modified with 2'-methoxy
  modified_base 1..3: mod_base = OTHER; note = two adjacent nucleosides are linked by phosphorothioate diester groups
  modified_base 19..21: mod_base = OTHER; note = two adjacent nucleosides are linked by phosphorothioate diester groups
  modified_base 1: mod_base = OTHER; note = 5'-E-VP
tccatcctcatcgtcctcgtc

SEQ ID NO: 187 - RNA, 21 nt, Synthetic Construct
  source 1..21: mol_type = other RNA; note = modified anti-sense strand
  modified_base 1: mod_base = OTHER; note = modified with 2'-methoxy
  modified_base 2: mod_base = OTHER; note = modified with 2'-Fluoro
  modified_base 3..5: mod_base = OTHER; note = modified with 2'-methoxy
  modified_base 6: mod_base = OTHER; note = modified with 2'-Fluoro
  modified_base 7..11: mod_base = OTHER; note = modified with 2'-methoxy
  modified_base 12: mod_base = OTHER; note = modified with 2'-Fluoro
  modified_base 13: mod_base = OTHER; note = modified with 2'-methoxy
  modified_base 14: mod_base = OTHER; note = modified with 2'-Fluoro
  modified_base 15: mod_base = OTHER; note = modified with 2'-methoxy
  modified_base 16: mod_base = OTHER; note = modified with 2'-Fluoro
  modified_base 17..21: mod_base = OTHER; note = modified with 2'-methoxy
  modified_base 1..3: mod_base = OTHER; note = two adjacent nucleosides are linked by phosphorothioate diester groups
  modified_base 19..21: mod_base = OTHER; note = two adjacent nucleosides are linked by phosphorothioate diester groups
  modified_base 1: mod_base = OTHER; note = 5'-E-VP
ttcaccatcctcatcgtcctc

SEQ ID NO: 188 - RNA, 21 nt, Synthetic Construct
  source 1..21: mol_type = other RNA; note = modified anti-sense strand
  modified_base 1: mod_base = OTHER; note = modified with 2'-methoxy
  modified_base 2: mod_base = OTHER; note = modified with 2'-Fluoro
  modified_base 3..5: mod_base = OTHER; note = modified with 2'-methoxy
  modified_base 6: mod_base = OTHER; note = modified with 2'-Fluoro
  modified_base 7..11: mod_base = OTHER; note = modified with 2'-methoxy
  modified_base 12: mod_base = OTHER; note = modified with 2'-Fluoro
  modified_base 13: mod_base = OTHER; note = modified with 2'-methoxy
  modified_base 14: mod_base = OTHER; note = modified with 2'-Fluoro
  modified_base 15: mod_base = OTHER; note = modified with 2'-methoxy
  modified_base 16: mod_base = OTHER; note = modified with 2'-Fluoro
  modified_base 17..21: mod_base = OTHER; note = modified with 2'-methoxy
  modified_base 1..3: mod_base = OTHER; note = two adjacent nucleosides are linked by phosphorothioate diester groups
  modified_base 19..21: mod_base = OTHER; note = two adjacent nucleosides are linked by phosphorothioate diester groups
  modified_base 1: mod_base = OTHER; note = 5'-E-VP
ttcatcaccatcctcatcgtc

SEQ ID NO: 189 - RNA, 21 nt, Synthetic Construct
  source 1..21: mol_type = other RNA; note = modified anti-sense strand
  modified_base 1: mod_base = OTHER; note = modified with 2'-methoxy
  modified_base 2: mod_base = OTHER; note = modified with 2'-Fluoro
  modified_base 3..5: mod_base = OTHER; note = modified with 2'-methoxy
  modified_base 6: mod_base = OTHER; note = modified with 2'-Fluoro
  modified_base 7..11: mod_base = OTHER; note = modified with 2'-methoxy
  modified_base 12: mod_base = OTHER; note = modified with 2'-Fluoro
  modified_base 13: mod_base = OTHER; note = modified with 2'-methoxy
  modified_base 14: mod_base = OTHER; note = modified with 2'-Fluoro
  modified_base 15: mod_base = OTHER; note = modified with 2'-methoxy
  modified_base 16: mod_base = OTHER; note = modified with 2'-Fluoro
  modified_base 17..21: mod_base = OTHER; note = modified with 2'-methoxy
  modified_base 1..3: mod_base = OTHER; note = two adjacent nucleosides are linked by phosphorothioate diester groups
  modified_base 19..21: mod_base = OTHER; note = two adjacent nucleosides are linked by phosphorothioate diester groups
  modified_base 1: mod_base = OTHER; note = 5'-E-VP
ttcgtagggttcctcagcctc

SEQ ID NO: 190 - RNA, 21 nt, Synthetic Construct
  source 1..21: mol_type = other RNA; note = modified anti-sense strand
  modified_base 1: mod_base = OTHER; note = modified with 2'-methoxy
  modified_base 2: mod_base = OTHER; note = modified with 2'-Fluoro
  modified_base 3..5: mod_base = OTHER; note = modified with 2'-methoxy
  modified_base 6: mod_base = OTHER; note = modified with 2'-Fluoro
  modified_base 7..11: mod_base = OTHER; note = modified with 2'-methoxy
  modified_base 12: mod_base = OTHER; note = modified with 2'-Fluoro
  modified_base 13: mod_base = OTHER; note = modified with 2'-methoxy
  modified_base 14: mod_base = OTHER; note = modified with 2'-Fluoro
  modified_base 15: mod_base = OTHER; note = modified with 2'-methoxy
  modified_base 16: mod_base = OTHER; note = modified with 2'-Fluoro
  modified_base 17..21: mod_base = OTHER; note = modified with 2'-methoxy
  modified_base 1..3: mod_base = OTHER; note = two adjacent nucleosides are linked by phosphorothioate diester groups
  modified_base 19..21: mod_base = OTHER; note = two adjacent nucleosides are linked by phosphorothioate diester groups
  modified_base 1: mod_base = OTHER; note = 5'-E-VP
tttcgtagggttcctcagcct

SEQ ID NO: 191 - RNA, 21 nt, Synthetic Construct
  source 1..21: mol_type = other RNA; note = modified anti-sense strand
  modified_base 1: mod_base = OTHER; note = modified with 2'-methoxy
  modified_base 2: mod_base = OTHER; note = modified with 2'-Fluoro
  modified_base 3..5: mod_base = OTHER; note = modified with 2'-methoxy
  modified_base 6: mod_base = OTHER; note = modified with 2'-Fluoro
  modified_base 7..11: mod_base = OTHER; note = modified with 2'-methoxy
  modified_base 12: mod_base = OTHER; note = modified with 2'-Fluoro
  modified_base 13: mod_base = OTHER; note = modified with 2'-methoxy
  modified_base 14: mod_base = OTHER; note = modified with 2'-Fluoro
  modified_base 15: mod_base = OTHER; note = modified with 2'-methoxy
  modified_base 16: mod_base = OTHER; note = modified with 2'-Fluoro
  modified_base 17..21: mod_base = OTHER; note = modified with 2'-methoxy
  modified_base 1..3: mod_base = OTHER; note = two adjacent nucleosides are linked by phosphorothioate diester groups
  modified_base 19..21: mod_base = OTHER; note = two adjacent nucleosides are linked by phosphorothioate diester groups
  modified_base 1: mod_base = OTHER; note = 5'-E-VP
tcttcgtagggttcctcagcc

SEQ ID NO: 192 - RNA, 21 nt, Synthetic Construct
  source 1..21: mol_type = other RNA; note = modified anti-sense strand
  modified_base 1: mod_base = OTHER; note = modified with 2'-methoxy
  modified_base 2: mod_base = OTHER; note = modified with 2'-Fluoro
  modified_base 3..5: mod_base = OTHER; note = modified with 2'-methoxy
  modified_base 6: mod_base = OTHER; note = modified with 2'-Fluoro
  modified_base 7..11: mod_base = OTHER; note = modified with 2'-methoxy
  modified_base 12: mod_base = OTHER; note = modified with 2'-Fluoro
  modified_base 13: mod_base = OTHER; note = modified with 2'-methoxy
  modified_base 14: mod_base = OTHER; note = modified with 2'-Fluoro
  modified_base 15: mod_base = OTHER; note = modified with 2'-methoxy
  modified_base 16: mod_base = OTHER; note = modified with 2'-Fluoro
  modified_base 17..21: mod_base = OTHER; note = modified with 2'-methoxy
  modified_base 1..3: mod_base = OTHER; note = two adjacent nucleosides are linked by phosphorothioate diester groups
  modified_base 19..21: mod_base = OTHER; note = two adjacent nucleosides are linked by phosphorothioate diester groups
  modified_base 1: mod_base = OTHER; note = 5'-E-VP
ttcttcgtagggttcctcagc

SEQ ID NO: 193 - RNA, 21 nt, Synthetic Construct
  source 1..21: mol_type = other RNA; note = modified anti-sense strand
  modified_base 1: mod_base = OTHER; note = modified with 2'-methoxy
  modified_base 2: mod_base = OTHER; note = modified with 2'-Fluoro
  modified_base 3..5: mod_base = OTHER; note = modified with 2'-methoxy
  modified_base 6: mod_base = OTHER; note = modified with 2'-Fluoro
  modified_base 7..11: mod_base = OTHER; note = modified with 2'-methoxy
  modified_base 12: mod_base = OTHER; note = modified with 2'-Fluoro
  modified_base 13: mod_base = OTHER; note = modified with 2'-methoxy
  modified_base 14: mod_base = OTHER; note = modified with 2'-Fluoro
  modified_base 15: mod_base = OTHER; note = modified with 2'-methoxy
  modified_base 16: mod_base = OTHER; note = modified with 2'-Fluoro
  modified_base 17..21: mod_base = OTHER; note = modified with 2'-methoxy
  modified_base 1..3: mod_base = OTHER; note = two adjacent nucleosides are linked by phosphorothioate diester groups
  modified_base 19..21: mod_base = OTHER; note = two adjacent nucleosides are linked by phosphorothioate diester groups
  modified_base 1: mod_base = OTHER; note = 5'-E-VP
tttcttcgtagggttcctcag

SEQ ID NO: 194 - RNA, 21 nt, Synthetic Construct
  source 1..21: mol_type = other RNA; note = modified anti-sense strand
  modified_base 1: mod_base = OTHER; note = modified with 2'-methoxy
  modified_base 2: mod_base = OTHER; note = modified with 2'-Fluoro
  modified_base 3..5: mod_base = OTHER; note = modified with 2'-methoxy
  modified_base 6: mod_base = OTHER; note = modified with 2'-Fluoro
  modified_base 7..11: mod_base = OTHER; note = modified with 2'-methoxy
  modified_base 12: mod_base = OTHER; note = modified with 2'-Fluoro
  modified_base 13: mod_base = OTHER; note = modified with 2'-methoxy
  modified_base 14: mod_base = OTHER; note = modified with 2'-Fluoro
  modified_base 15: mod_base = OTHER; note = modified with 2'-methoxy
  modified_base 16: mod_base = OTHER; note = modified with 2'-Fluoro
  modified_base 17..21: mod_base = OTHER; note = modified with 2'-methoxy
  modified_base 1..3: mod_base = OTHER; note = two adjacent nucleosides are linked by phosphorothioate diester groups
  modified_base 19..21: mod_base = OTHER; note = two adjacent nucleosides are linked by phosphorothioate diester groups
  modified_base 1: mod_base = OTHER; note = 5'-E-VP
tggcttcttcgtagggttcct

SEQ ID NO: 195 - RNA, 21 nt, Synthetic Construct
  source 1..21: mol_type = other RNA; note = modified anti-sense strand
  modified_base 1: mod_base = OTHER; note = modified with 2'-methoxy
  modified_base 2: mod_base = OTHER; note = modified with 2'-Fluoro
  modified_base 3..5: mod_base = OTHER; note = modified with 2'-methoxy
  modified_base 6: mod_base = OTHER; note = modified with 2'-Fluoro
  modified_base 7..11: mod_base = OTHER; note = modified with 2'-methoxy
  modified_base 12: mod_base = OTHER; note = modified with 2'-Fluoro
  modified_base 13: mod_base = OTHER; note = modified with 2'-methoxy
  modified_base 14: mod_base = OTHER; note = modified with 2'-Fluoro
  modified_base 15: mod_base = OTHER; note = modified with 2'-methoxy
  modified_base 16: mod_base = OTHER; note = modified with 2'-Fluoro
  modified_base 17..21: mod_base = OTHER; note = modified with 2'-methoxy
  modified_base 1..3: mod_base = OTHER; note = two adjacent nucleosides are linked by phosphorothioate diester groups
  modified_base 19..21: mod_base = OTHER; note = two adjacent nucleosides are linked by phosphorothioate diester groups
  modified_base 1: mod_base = OTHER; note = 5'-E-VP
tgtggcttcttcgtagggttc

SEQ ID NO: 196 - RNA, 21 nt, Synthetic Construct
  source 1..21: mol_type = other RNA; note = modified anti-sense strand
  modified_base 1: mod_base = OTHER; note = modified with 2'-methoxy
  modified_base 2: mod_base = OTHER; note = modified with 2'-Fluoro
  modified_base 3..5: mod_base = OTHER; note = modified with 2'-methoxy
  modified_base 6: mod_base = OTHER; note = modified with 2'-Fluoro
  modified_base 7..11: mod_base = OTHER; note = modified with 2'-methoxy
  modified_base 12: mod_base = OTHER; note = modified with 2'-Fluoro
  modified_base 13: mod_base = OTHER; note = modified with 2'-methoxy
  modified_base 14: mod_base = OTHER; note = modified with 2'-Fluoro
  modified_base 15: mod_base = OTHER; note = modified with 2'-methoxy
  modified_base 16: mod_base = OTHER; note = modified with 2'-Fluoro
  modified_base 17..21: mod_base = OTHER; note = modified with 2'-methoxy
  modified_base 1..3: mod_base = OTHER; note = two adjacent nucleosides are linked by phosphorothioate diester groups
  modified_base 19..21: mod_base = OTHER; note = two adjacent nucleosides are linked by phosphorothioate diester groups
  modified_base 1: mod_base = OTHER; note = 5'-E-VP
tctgtggcttcttcgtagggt

SEQ ID NO: 197 - RNA, 21 nt, Synthetic Construct
  source 1..21: mol_type = other RNA; note = modified anti-sense strand
  modified_base 1: mod_base = OTHER; note = modified with 2'-methoxy
  modified_base 2: mod_base = OTHER; note = modified with 2'-Fluoro
  modified_base 3..5: mod_base = OTHER; note = modified with 2'-methoxy
  modified_base 6: mod_base = OTHER; note = modified with 2'-Fluoro
  modified_base 7..11: mod_base = OTHER; note = modified with 2'-methoxy
  modified_base 12: mod_base = OTHER; note = modified with 2'-Fluoro
  modified_base 13: mod_base = OTHER; note = modified with 2'-methoxy
  modified_base 14: mod_base = OTHER; note = modified with 2'-Fluoro
  modified_base 15: mod_base = OTHER; note = modified with 2'-methoxy
  modified_base 16: mod_base = OTHER; note = modified with 2'-Fluoro
  modified_base 17..21: mod_base = OTHER; note = modified with 2'-methoxy
  modified_base 1..3: mod_base = OTHER; note = two adjacent nucleosides are linked by phosphorothioate diester groups
  modified_base 19..21: mod_base = OTHER; note = two adjacent nucleosides are linked by phosphorothioate diester groups
  modified_base 1: mod_base = OTHER; note = 5'-E-VP
tctctgtggcttcttcgtagg

SEQ ID NO: 198 - RNA, 21 nt, Synthetic Construct
  source 1..21: mol_type = other RNA; note = modified anti-sense strand
  modified_base 1: mod_base = OTHER; note = modified with 2'-methoxy
  modified_base 2: mod_base = OTHER; note = modified with 2'-Fluoro
  modified_base 3..5: mod_base = OTHER; note = modified with 2'-methoxy
  modified_base 6: mod_base = OTHER; note = modified with 2'-Fluoro
  modified_base 7..11: mod_base = OTHER; note = modified with 2'-methoxy
  modified_base 12: mod_base = OTHER; note = modified with 2'-Fluoro
  modified_base 13: mod_base = OTHER; note = modified with 2'-methoxy
  modified_base 14: mod_base = OTHER; note = modified with 2'-Fluoro
  modified_base 15: mod_base = OTHER; note = modified with 2'-methoxy
  modified_base 16: mod_base = OTHER; note = modified with 2'-Fluoro
  modified_base 17..21: mod_base = OTHER; note = modified with 2'-methoxy
  modified_base 1..3: mod_base = OTHER; note = two adjacent nucleosides are linked by phosphorothioate diester groups
  modified_base 19..21: mod_base = OTHER; note = two adjacent nucleosides are linked by phosphorothioate diester groups
  modified_base 1: mod_base = OTHER; note = 5'-E-VP
tctctctgtggcttcttcgta

SEQ ID NO: 199 - RNA, 21 nt, Synthetic Construct
  source 1..21: mol_type = other RNA; note = modified anti-sense strand
  modified_base 1: mod_base = OTHER; note = modified with 2'-methoxy
  modified_base 2: mod_base = OTHER; note = modified with 2'-Fluoro
  modified_base 3..5: mod_base = OTHER; note = modified with 2'-methoxy
  modified_base 6: mod_base = OTHER; note = modified with 2'-Fluoro
  modified_base 7..11: mod_base = OTHER; note = modified with 2'-methoxy
  modified_base 12: mod_base = OTHER; note = modified with 2'-Fluoro
  modified_base 13: mod_base = OTHER; note = modified with 2'-methoxy
  modified_base 14: mod_base = OTHER; note = modified with 2'-Fluoro
  modified_base 15: mod_base = OTHER; note = modified with 2'-methoxy
  modified_base 16: mod_base = OTHER; note = modified with 2'-Fluoro
  modified_base 17..21: mod_base = OTHER; note = modified with 2'-methoxy
  modified_base 1..3: mod_base = OTHER; note = two adjacent nucleosides are linked by phosphorothioate diester groups
  modified_base 19..21: mod_base = OTHER; note = two adjacent nucleosides are linked by phosphorothioate diester groups
  modified_base 1: mod_base = OTHER; note = 5'-E-VP
ttctctctgtggcttcttcgt

SEQ ID NO: 200 - RNA, 21 nt, Synthetic Construct
  source 1..21: mol_type = other RNA; note = modified anti-sense strand
  modified_base 1: mod_base = OTHER; note = modified with 2'-methoxy
  modified_base 2: mod_base = OTHER; note = modified with 2'-Fluoro
  modified_base 3..5: mod_base = OTHER; note = modified with 2'-methoxy
  modified_base 6: mod_base = OTHER; note = modified with 2'-Fluoro
  modified_base 7..11: mod_base = OTHER; note = modified with 2'-methoxy
  modified_base 12: mod_base = OTHER; note = modified with 2'-Fluoro
  modified_base 13: mod_base = OTHER; note = modified with 2'-methoxy
  modified_base 14: mod_base = OTHER; note = modified with 2'-Fluoro
  modified_base 15: mod_base = OTHER; note = modified with 2'-methoxy
  modified_base 16: mod_base = OTHER; note = modified with 2'-Fluoro
  modified_base 17..21: mod_base = OTHER; note = modified with 2'-methoxy
  modified_base 1..3: mod_base = OTHER; note = two adjacent nucleosides are linked by phosphorothioate diester groups
  modified_base 19..21: mod_base = OTHER; note = two adjacent nucleosides are linked by phosphorothioate diester groups
  modified_base 1: mod_base = OTHER; note = 5'-E-VP
tggttctctctgtggcttctt

SEQ ID NO: 201 - RNA, 21 nt, Synthetic Construct
  source 1..21: mol_type = other RNA; note = modified anti-sense strand
  modified_base 1: mod_base = OTHER; note = modified with 2'-methoxy
  modified_base 2: mod_base = OTHER; note = modified with 2'-Fluoro
  modified_base 3..5: mod_base = OTHER; note = modified with 2'-methoxy
  modified_base 6: mod_base = OTHER; note = modified with 2'-Fluoro
  modified_base 7..11: mod_base = OTHER; note = modified with 2'-methoxy
  modified_base 12: mod_base = OTHER; note = modified with 2'-Fluoro
  modified_base 13: mod_base = OTHER; note = modified with 2'-methoxy
  modified_base 14: mod_base = OTHER; note = modified with 2'-Fluoro
  modified_base 15: mod_base = OTHER; note = modified with 2'-methoxy
  modified_base 16: mod_base = OTHER; note = modified with 2'-Fluoro
  modified_base 17..21: mod_base = OTHER; note = modified with 2'-methoxy
  modified_base 1..3: mod_base = OTHER; note = two adjacent nucleosides are linked by phosphorothioate diester groups
  modified_base 19..21: mod_base = OTHER; note = two adjacent nucleosides are linked by phosphorothioate diester groups
  modified_base 1: mod_base = OTHER; note = 5'-E-VP
tggtggttctctctgtggctt

SEQ ID NO: 202 - RNA, 21 nt, Synthetic Construct
  source 1..21: mol_type = other RNA; note = modified anti-sense strand
  modified_base 1: mod_base = OTHER; note = modified with 2'-methoxy
  modified_base 2: mod_base = OTHER; note = modified with 2'-Fluoro
  modified_base 3..5: mod_base = OTHER; note = modified with 2'-methoxy
  modified_base 6: mod_base = OTHER; note = modified with 2'-Fluoro
  modified_base 7..11: mod_base = OTHER; note = modified with 2'-methoxy
  modified_base 12: mod_base = OTHER; note = modified with 2'-Fluoro
  modified_base 13: mod_base = OTHER; note = modified with 2'-methoxy
  modified_base 14: mod_base = OTHER; note = modified with 2'-Fluoro
  modified_base 15: mod_base = OTHER; note = modified with 2'-methoxy
  modified_base 16: mod_base = OTHER; note = modified with 2'-Fluoro
  modified_base 17..21: mod_base = OTHER; note = modified with 2'-methoxy
  modified_base 1..3: mod_base = OTHER; note = two adjacent nucleosides are linked by phosphorothioate diester groups
  modified_base 19..21: mod_base = OTHER; note = two adjacent nucleosides are linked by phosphorothioate diester groups
  modified_base 1: mod_base = OTHER; note = 5'-E-VP
ttggtggttctctctgtggct

SEQ ID NO: 203 - RNA, 21 nt, Synthetic Construct
  source 1..21: mol_type = other RNA; note = modified anti-sense strand
  modified_base 1: mod_base = OTHER; note = modified with 2'-methoxy
  modified_base 2: mod_base = OTHER; note = modified with 2'-Fluoro
  modified_base 3..5: mod_base = OTHER; note = modified with 2'-methoxy
  modified_base 6: mod_base = OTHER; note = modified with 2'-Fluoro
  modified_base 7..11: mod_base = OTHER; note = modified with 2'-methoxy
  modified_base 12: mod_base = OTHER; note = modified with 2'-Fluoro
  modified_base 13: mod_base = OTHER; note = modified with 2'-methoxy
  modified_base 14: mod_base = OTHER; note = modified with 2'-Fluoro
  modified_base 15: mod_base = OTHER; note = modified with 2'-methoxy
  modified_base 16: mod_base = OTHER; note = modified with 2'-Fluoro
  modified_base 17..21: mod_base = OTHER; note = modified with 2'-methoxy
  modified_base 1..3: mod_base = OTHER; note = two adjacent nucleosides are linked by phosphorothioate diester groups
  modified_base 19..21: mod_base = OTHER; note = two adjacent nucleosides are linked by phosphorothioate diester groups
  modified_base 1: mod_base = OTHER; note = 5'-E-VP
tggtggtggtggtggtggcaa

SEQ ID NO: 204 - RNA, 21 nt, Synthetic Construct
  source 1..21: mol_type = other RNA; note = modified anti-sense strand
  modified_base 1: mod_base = OTHER; note = modified with 2'-methoxy
  modified_base 2: mod_base = OTHER; note = modified with 2'-Fluoro
  modified_base 3..5: mod_base = OTHER; note = modified with 2'-methoxy
  modified_base 6: mod_base = OTHER; note = modified with 2'-Fluoro
  modified_base 7..11: mod_base = OTHER; note = modified with 2'-methoxy
  modified_base 12: mod_base = OTHER; note = modified with 2'-Fluoro
  modified_base 13: mod_base = OTHER; note = modified with 2'-methoxy
  modified_base 14: mod_base = OTHER; note = modified with 2'-Fluoro
  modified_base 15: mod_base = OTHER; note = modified with 2'-methoxy
  modified_base 16: mod_base = OTHER; note = modified with 2'-Fluoro
  modified_base 17..21: mod_base = OTHER; note = modified with 2'-methoxy
  modified_base 1..3: mod_base = OTHER; note = two adjacent nucleosides are linked by phosphorothioate diester groups
  modified_base 19..21: mod_base = OTHER; note = two adjacent nucleosides are linked by phosphorothioate diester groups
  modified_base 1: mod_base = OTHER; note = 5'-E-VP
tgttcagagcacacctctcga

SEQ ID NO: 205 - RNA, 21 nt, Synthetic Construct
  source 1..21: mol_type = other RNA; note = modified anti-sense strand
  modified_base 1: mod_base = OTHER; note = modified with 2'-methoxy
  modified_base 2: mod_base = OTHER; note = modified with 2'-Fluoro
  modified_base 3..5: mod_base = OTHER; note = modified with 2'-methoxy
  modified_base 6: mod_base = OTHER; note = modified with 2'-Fluoro
  modified_base 7..11: mod_base = OTHER; note = modified with 2'-methoxy
  modified_base 12: mod_base = OTHER; note = modified with 2'-Fluoro
  modified_base 13: mod_base = OTHER; note = modified with 2'-methoxy
  modified_base 14: mod_base = OTHER; note = modified with 2'-Fluoro
  modified_base 15: mod_base = OTHER; note = modified with 2'-methoxy
  modified_base 16: mod_base = OTHER; note = modified with 2'-Fluoro
  modified_base 17..21: mod_base = OTHER; note = modified with 2'-methoxy
  modified_base 1..3: mod_base = OTHER; note = two adjacent nucleosides are linked by phosphorothioate diester groups
  modified_base 19..21: mod_base = OTHER; note = two adjacent nucleosides are linked by phosphorothioate diester groups
  modified_base 1: mod_base = OTHER; note = 5'-E-VP
ttgttcagagcacacctctcg

SEQ ID NO: 206 - RNA, 21 nt, Synthetic Construct
  source 1..21: mol_type = other RNA; note = modified anti-sense strand
  modified_base 1: mod_base = OTHER; note = modified with 2'-methoxy
  modified_base 2: mod_base = OTHER; note = modified with 2'-Fluoro
  modified_base 3..5: mod_base = OTHER; note = modified with 2'-methoxy
  modified_base 6: mod_base = OTHER; note = modified with 2'-Fluoro
  modified_base 7..11: mod_base = OTHER; note = modified with 2'-methoxy
  modified_base 12: mod_base = OTHER; note = modified with 2'-Fluoro
  modified_base 13: mod_base = OTHER; note = modified with 2'-methoxy
  modified_base 14: mod_base = OTHER; note = modified with 2'-Fluoro
  modified_base 15: mod_base = OTHER; note = modified with 2'-methoxy
  modified_base 16: mod_base = OTHER; note = modified with 2'-Fluoro
  modified_base 17..21: mod_base = OTHER; note = modified with 2'-methoxy
  modified_base 1..3: mod_base = OTHER; note = two adjacent nucleosides are linked by phosphorothioate diester groups
  modified_base 19..21: mod_base = OTHER; note = two adjacent nucleosides are linked by phosphorothioate diester groups
  modified_base 1: mod_base = OTHER; note = 5'-E-VP
ttcattgctcggcacggcccc

SEQ ID NO: 207 - RNA, 21 nt, Synthetic Construct
  source 1..21: mol_type = other RNA; note = modified anti-sense strand
  modified_base 1: mod_base = OTHER; note = modified with 2'-methoxy
  modified_base 2: mod_base = OTHER; note = modified with 2'-Fluoro
  modified_base 3..5: mod_base = OTHER; note = modified with 2'-methoxy
  modified_base 6: mod_base = OTHER; note = modified with 2'-Fluoro
  modified_base 7..11: mod_base = OTHER; note = modified with 2'-methoxy
  modified_base 12: mod_base = OTHER; note = modified with 2'-Fluoro
  modified_base 13: mod_base = OTHER; note = modified with 2'-methoxy
  modified_base 14: mod_base = OTHER; note = modified with 2'-Fluoro
  modified_base 15: mod_base = OTHER; note = modified with 2'-methoxy
  modified_base 16: mod_base = OTHER; note = modified with 2'-Fluoro
  modified_base 17..21: mod_base = OTHER; note = modified with 2'-methoxy
  modified_base 1..3: mod_base = OTHER; note = two adjacent nucleosides are linked by phosphorothioate diester groups
  modified_base 19..21: mod_base = OTHER; note = two adjacent nucleosides are linked by phosphorothioate diester groups
  modified_base 1: mod_base = OTHER; note = 5'-E-VP
tgatcattgctcggcacggcc

SEQ ID NO: 208 - RNA, 21 nt, Synthetic Construct
  source 1..21: mol_type = other RNA; note = modified anti-sense strand
  modified_base 1: mod_base = OTHER; note = modified with 2'-methoxy
  modified_base 2: mod_base = OTHER; note = modified with 2'-Fluoro
  modified_base 3..5: mod_base = OTHER; note = modified with 2'-methoxy
  modified_base 6: mod_base = OTHER; note = modified with 2'-Fluoro
  modified_base 7..11: mod_base = OTHER; note = modified with 2'-methoxy
  modified_base 12: mod_base = OTHER; note = modified with 2'-Fluoro
  modified_base 13: mod_base = OTHER; note = modified with 2'-methoxy
  modified_base 14: mod_base = OTHER; note = modified with 2'-Fluoro
  modified_base 15: mod_base = OTHER; note = modified with 2'-methoxy
  modified_base 16: mod_base = OTHER; note = modified with 2'-Fluoro
  modified_base 17..21: mod_base = OTHER; note = modified with 2'-methoxy
  modified_base 1..3: mod_base = OTHER; note = two adjacent nucleosides are linked by phosphorothioate diester groups
  modified_base 19..21: mod_base = OTHER; note = two adjacent nucleosides are linked by phosphorothioate diester groups
  modified_base 1: mod_base = OTHER; note = 5'-E-VP
tagatcattgctcggcacggc

SEQ ID NO: 209 - RNA, 21 nt, Synthetic Construct
  source 1..21: mol_type = other RNA; note = modified anti-sense strand
  modified_base 1: mod_base = OTHER; note = modified with 2'-methoxy
  modified_base 2: mod_base = OTHER; note = modified with 2'-Fluoro
  modified_base 3..5: mod_base = OTHER; note = modified with 2'-methoxy
  modified_base 6: mod_base = OTHER; note = modified with 2'-Fluoro
  modified_base 7..11: mod_base = OTHER; note = modified with 2'-methoxy
  modified_base 12: mod_base = OTHER; note = modified with 2'-Fluoro
  modified_base 13: mod_base = OTHER; note = modified with 2'-methoxy
  modified_base 14: mod_base = OTHER; note = modified with 2'-Fluoro
  modified_base 15: mod_base = OTHER; note = modified with 2'-methoxy
  modified_base 16: mod_base = OTHER; note = modified with 2'-Fluoro
  modified_base 17..21: mod_base = OTHER; note = modified with 2'-methoxy
  modified_base 1..3: mod_base = OTHER; note = two adjacent nucleosides are linked by phosphorothioate diester groups
  modified_base 19..21: mod_base = OTHER; note = two adjacent nucleosides are linked by phosphorothioate diester groups
  modified_base 1: mod_base = OTHER; note = 5'-E-VP
tccggttgccgccacatccgc

SEQ ID NO: 210 - RNA, 21 nt, Synthetic Construct
  source 1..21: mol_type = other RNA; note = modified anti-sense strand
  modified_base 1: mod_base = OTHER; note = modified with 2'-methoxy
  modified_base 2: mod_base = OTHER; note = modified with 2'-Fluoro
  modified_base 3..5: mod_base = OTHER; note = modified with 2'-methoxy
  modified_base 6: mod_base = OTHER; note = modified with 2'-Fluoro
  modified_base 7..11: mod_base = OTHER; note = modified with 2'-methoxy
  modified_base 12: mod_base = OTHER; note = modified with 2'-Fluoro
  modified_base 13: mod_base = OTHER; note = modified with 2'-methoxy
  modified_base 14: mod_base = OTHER; note = modified with 2'-Fluoro
  modified_base 15: mod_base = OTHER; note = modified with 2'-methoxy
  modified_base 16: mod_base = OTHER; note = modified with 2'-Fluoro
  modified_base 17..21: mod_base = OTHER; note = modified with 2'-methoxy
  modified_base 1..3: mod_base = OTHER; note = two adjacent nucleosides are linked by phosphorothioate diester groups
  modified_base 19..21: mod_base = OTHER; note = two adjacent nucleosides are linked by phosphorothioate diester groups
  modified_base 1: mod_base = OTHER; note = 5'-E-VP
ttccggttgccgccacatccg

SEQ ID NO: 211 - RNA, 21 nt, Synthetic Construct
  source 1..21: mol_type = other RNA; note = modified anti-sense strand
  modified_base 1: mod_base = OTHER; note = modified with 2'-methoxy
  modified_base 2: mod_base = OTHER; note = modified with 2'-Fluoro
  modified_base 3..5: mod_base = OTHER; note = modified with 2'-methoxy
  modified_base 6: mod_base = OTHER; note = modified with 2'-Fluoro
  modified_base 7..11: mod_base = OTHER; note = modified with 2'-methoxy
  modified_base 12: mod_base = OTHER; note = modified with 2'-Fluoro
  modified_base 13: mod_base = OTHER; note = modified with 2'-methoxy
  modified_base 14: mod_base = OTHER; note = modified with 2'-Fluoro
  modified_base 15: mod_base = OTHER; note = modified with 2'-methoxy
  modified_base 16: mod_base = OTHER; note = modified with 2'-Fluoro
  modified_base 17..21: mod_base = OTHER; note = modified with 2'-methoxy
  modified_base 1..3: mod_base = OTHER; note = two adjacent nucleosides are linked by phosphorothioate diester groups
  modified_base 19..21: mod_base = OTHER; note = two adjacent nucleosides are linked by phosphorothioate diester groups
  modified_base 1: mod_base = OTHER; note = 5'-E-VP
tgttgttccggttgccgccac

SEQ ID NO: 212 - RNA, 21 nt, Synthetic Construct
  source 1..21: mol_type = other RNA; note = modified anti-sense strand
  modified_base 1: mod_base = OTHER; note = modified with 2'-methoxy
  modified_base 2: mod_base = OTHER; note = modified with 2'-Fluoro
  modified_base 3..5: mod_base = OTHER; note = modified with 2'-methoxy
  modified_base 6: mod_base = OTHER; note = modified with 2'-Fluoro
  modified_base 7..11: mod_base = OTHER; note = modified with 2'-methoxy
  modified_base 12: mod_base = OTHER; note = modified with 2'-Fluoro
  modified_base 13: mod_base = OTHER; note = modified with 2'-methoxy
  modified_base 14: mod_base = OTHER; note = modified with 2'-Fluoro
  modified_base 15: mod_base = OTHER; note = modified with 2'-methoxy
  modified_base 16: mod_base = OTHER; note = modified with 2'-Fluoro
  modified_base 17..21: mod_base = OTHER; note = modified with 2'-methoxy
  modified_base 1..3: mod_base = OTHER; note = two adjacent nucleosides are linked by phosphorothioate diester groups
  modified_base 19..21: mod_base = OTHER; note = two adjacent nucleosides are linked by phosphorothioate diester groups
  modified_base 1: mod_base = OTHER; note = 5'-E-VP
tagttgttccggttgccgcca

SEQ ID NO: 213 - RNA, 21 nt, Synthetic Construct
  source 1..21: mol_type = other RNA; note = modified anti-sense strand
  modified_base 1: mod_base = OTHER; note = modified with 2'-methoxy
  modified_base 2: mod_base = OTHER; note = modified with 2'-Fluoro
  modified_base 3..5: mod_base = OTHER; note = modified with 2'-methoxy
  modified_base 6: mod_base = OTHER; note = modified with 2'-Fluoro
  modified_base 7..11: mod_base = OTHER; note = modified with 2'-methoxy
  modified_base 12: mod_base = OTHER; note = modified with 2'-Fluoro
  modified_base 13: mod_base = OTHER; note = modified with 2'-methoxy
  modified_base 14: mod_base = OTHER; note = modified with 2'-Fluoro
  modified_base 15: mod_base = OTHER; note = modified with 2'-methoxy
  modified_base 16: mod_base = OTHER; note = modified with 2'-Fluoro
  modified_base 17..21: mod_base = OTHER; note = modified with 2'-methoxy
  modified_base 1..3: mod_base = OTHER; note = two adjacent nucleosides are linked by phosphorothioate diester groups
  modified_base 19..21: mod_base = OTHER; note = two adjacent nucleosides are linked by phosphorothioate diester groups
  modified_base 1: mod_base = OTHER; note = 5'-E-VP
taagttgttccggttgccgcc

SEQ ID NO: 214 - RNA, 21 nt, Synthetic Construct
  source 1..21: mol_type = other RNA; note = modified anti-sense strand
  modified_base 1: mod_base = OTHER; note = modified with 2'-methoxy
  modified_base 2: mod_base = OTHER; note = modified with 2'-Fluoro
  modified_base 3..5: mod_base = OTHER; note = modified with 2'-methoxy
  modified_base 6: mod_base = OTHER; note = modified with 2'-Fluoro
  modified_base 7..11: mod_base = OTHER; note = modified with 2'-methoxy
  modified_base 12: mod_base = OTHER; note = modified with 2'-Fluoro
  modified_base 13: mod_base = OTHER; note = modified with 2'-methoxy
  modified_base 14: mod_base = OTHER; note = modified with 2'-Fluoro
  modified_base 15: mod_base = OTHER; note = modified with 2'-methoxy
  modified_base 16: mod_base = OTHER; note = modified with 2'-Fluoro
  modified_base 17..21: mod_base = OTHER; note = modified with 2'-methoxy
  modified_base 1..3: mod_base = OTHER; note = two adjacent nucleosides are linked by phosphorothioate diester groups
  modified_base 19..21: mod_base = OTHER; note = two adjacent nucleosides are linked by phosphorothioate diester groups
  modified_base 1: mod_base = OTHER; note = 5'-E-VP
taaagttgttccggttgccgc

SEQ ID NO: 215 - RNA, 21 nt, Synthetic Construct
  source 1..21: mol_type = other RNA; note = modified anti-sense strand
  modified_base 1: mod_base = OTHER; note = modified with 2'-methoxy
  modified_base 2: mod_base = OTHER; note = modified with 2'-Fluoro
  modified_base 3..5: mod_base = OTHER; note = modified with 2'-methoxy
  modified_base 6: mod_base = OTHER; note = modified with 2'-Fluoro
  modified_base 7..11: mod_base = OTHER; note = modified with 2'-methoxy
  modified_base 12: mod_base = OTHER; note = modified with 2'-Fluoro
  modified_base 13: mod_base = OTHER; note = modified with 2'-methoxy
  modified_base 14: mod_base = OTHER; note = modified with 2'-Fluoro
  modified_base 15: mod_base = OTHER; note = modified with 2'-methoxy
  modified_base 16: mod_base = OTHER; note = modified with 2'-Fluoro
  modified_base 17..21: mod_base = OTHER; note = modified with 2'-methoxy
  modified_base 1..3: mod_base = OTHER; note = two adjacent nucleosides are linked by phosphorothioate diester groups
  modified_base 19..21: mod_base = OTHER; note = two adjacent nucleosides are linked by phosphorothioate diester groups
  modified_base 1: mod_base = OTHER; note = 5'-E-VP
tcaaagttgttccggttgccg

SEQ ID NO: 216 - RNA, 21 nt, Synthetic Construct
  source 1..21: mol_type = other RNA; note = modified anti-sense strand
  modified_base 1: mod_base = OTHER; note = modified with 2'-methoxy
  modified_base 2: mod_base = OTHER; note = modified with 2'-Fluoro
  modified_base 3..5: mod_base = OTHER; note = modified with 2'-methoxy
  modified_base 6: mod_base = OTHER; note = modified with 2'-Fluoro
  modified_base 7..11: mod_base = OTHER; note = modified with 2'-methoxy
  modified_base 12: mod_base = OTHER; note = modified with 2'-Fluoro
  modified_base 13: mod_base = OTHER; note = modified with 2'-methoxy
  modified_base 14: mod_base = OTHER; note = modified with 2'-Fluoro
  modified_base 15: mod_base = OTHER; note = modified with 2'-methoxy
  modified_base 16: mod_base = OTHER; note = modified with 2'-Fluoro
  modified_base 17..21: mod_base = OTHER; note = modified with 2'-methoxy
  modified_base 1..3: mod_base = OTHER; note = two adjacent nucleosides are linked by phosphorothioate diester groups
  modified_base 19..21: mod_base = OTHER; note = two adjacent nucleosides are linked by phosphorothioate diester groups
  modified_base 1: mod_base = OTHER; note = 5'-E-VP
tttctttgcttgacgttctgc

SEQ ID NO: 217 - RNA, 21 nt, Synthetic Construct
  source 1..21: mol_type = other RNA; note = modified anti-sense strand
  modified_base 1: mod_base = OTHER; note = modified with 2'-methoxy
  modified_base 2: mod_base = OTHER; note = modified with 2'-Fluoro
  modified_base 3..5: mod_base = OTHER; note = modified with 2'-methoxy
  modified_base 6: mod_base = OTHER; note = modified with 2'-Fluoro
  modified_base 7..11: mod_base = OTHER; note = modified with 2'-methoxy
  modified_base 12: mod_base = OTHER; note = modified with 2'-Fluoro
  modified_base 13: mod_base = OTHER; note = modified with 2'-methoxy
  modified_base 14: mod_base = OTHER; note = modified with 2'-Fluoro
  modified_base 15: mod_base = OTHER; note = modified with 2'-methoxy
  modified_base 16: mod_base = OTHER; note = modified with 2'-Fluoro
  modified_base 17..21: mod_base = OTHER; note = modified with 2'-methoxy
  modified_base 1..3: mod_base = OTHER; note = two adjacent nucleosides are linked by phosphorothioate diester groups
  modified_base 19..21: mod_base = OTHER; note = two adjacent nucleosides are linked by phosphorothioate diester groups
  modified_base 1: mod_base = OTHER; note = 5'-E-VP
tatggcttccactctggccat

SEQ ID NO: 218 - RNA, 21 nt, Synthetic Construct
  source 1..21: mol_type = other RNA; note = modified anti-sense strand
  modified_base 1: mod_base = OTHER; note = modified with 2'-methoxy
  modified_base 2: mod_base = OTHER; note = modified with 2'-Fluoro
  modified_base 3..5: mod_base = OTHER; note = modified with 2'-methoxy
  modified_base 6: mod_base = OTHER; note = modified with 2'-Fluoro
  modified_base 7..11: mod_base = OTHER; note = modified with 2'-methoxy
  modified_base 12: mod_base = OTHER; note = modified with 2'-Fluoro
  modified_base 13: mod_base = OTHER; note = modified with 2'-methoxy
  modified_base 14: mod_base = OTHER; note = modified with 2'-Fluoro
  modified_base 15: mod_base = OTHER; note = modified with 2'-methoxy
  modified_base 16: mod_base = OTHER; note = modified with 2'-Fluoro
  modified_base 17..21: mod_base = OTHER; note = modified with 2'-methoxy
  modified_base 1..3: mod_base = OTHER; note = two adjacent nucleosides are linked by phosphorothioate diester groups
  modified_base 19..21: mod_base = OTHER; note = two adjacent nucleosides are linked by phosphorothioate diester groups
  modified_base 1: mod_base = OTHER; note = 5'-E-VP
ttgtctgtccttctgttctgc

SEQ ID NO: 219 - RNA, 21 nt, Synthetic Construct
  source 1..21: mol_type = other RNA; note = modified anti-sense strand
  modified_base 1: mod_base = OTHER; note = modified with 2'-methoxy
  modified_base 2: mod_base = OTHER; note = modified with 2'-Fluoro
  modified_base 3..5: mod_base = OTHER; note = modified with 2'-methoxy
  modified_base 6: mod_base = OTHER; note = modified with 2'-Fluoro
  modified_base 7..11: mod_base = OTHER; note = modified with 2'-methoxy
  modified_base 12: mod_base = OTHER; note = modified with 2'-Fluoro
  modified_base 13: mod_base = OTHER; note = modified with 2'-methoxy
  modified_base 14: mod_base = OTHER; note = modified with 2'-Fluoro
  modified_base 15: mod_base = OTHER; note = modified with 2'-methoxy
  modified_base 16: mod_base = OTHER; note = modified with 2'-Fluoro
  modified_base 17..21: mod_base = OTHER; note = modified with 2'-methoxy
  modified_base 1..3: mod_base = OTHER; note = two adjacent nucleosides are linked by phosphorothioate diester groups
  modified_base 19..21: mod_base = OTHER; note = two adjacent nucleosides are linked by phosphorothioate diester groups
  modified_base 1: mod_base = OTHER; note = 5'-E-VP
tggctaaggggctatgtgata

SEQ ID NO: 220 - RNA, 21 nt, Synthetic Construct
  source 1..21: mol_type = other RNA; note = modified anti-sense strand
  modified_base 1: mod_base = OTHER; note = modified with 2'-methoxy
  modified_base 2: mod_base = OTHER; note = modified with 2'-Fluoro
  modified_base 3..5: mod_base = OTHER; note = modified with 2'-methoxy
  modified_base 6: mod_base = OTHER; note = modified with 2'-Fluoro
  modified_base 7..11: mod_base = OTHER; note = modified with 2'-methoxy
  modified_base 12: mod_base = OTHER; note = modified with 2'-Fluoro
  modified_base 13: mod_base = OTHER; note = modified with 2'-methoxy
  modified_base 14: mod_base = OTHER; note = modified with 2'-Fluoro
  modified_base 15: mod_base = OTHER; note = modified with 2'-methoxy
  modified_base 16: mod_base = OTHER; note = modified with 2'-Fluoro
  modified_base 17..21: mod_base = OTHER; note = modified with 2'-methoxy
  modified_base 1..3: mod_base = OTHER; note = two adjacent nucleosides are linked by phosphorothioate diester groups
  modified_base 19..21: mod_base = OTHER; note = two adjacent nucleosides are linked by phosphorothioate diester groups
  modified_base 1: mod_base = OTHER; note = 5'-E-VP
ttacaactggctaaggggcta

SEQ ID NO: 221 - RNA, 21 nt, Synthetic Construct
  source 1..21: mol_type = other RNA; note = modified anti-sense strand
  modified_base 1: mod_base = OTHER; note = modified with 2'-methoxy
  modified_base 2: mod_base = OTHER; note = modified with 2'-Fluoro
  modified_base 3..5: mod_base = OTHER; note = modified with 2'-methoxy
  modified_base 6: mod_base = OTHER; note = modified with 2'-Fluoro
  modified_base 7..11: mod_base = OTHER; note = modified with 2'-methoxy
  modified_base 12: mod_base = OTHER; note = modified with 2'-Fluoro
  modified_base 13: mod_base = OTHER; note = modified with 2'-methoxy
  modified_base 14: mod_base = OTHER; note = modified with 2'-Fluoro
  modified_base 15: mod_base = OTHER; note = modified with 2'-methoxy
  modified_base 16: mod_base = OTHER; note = modified with 2'-Fluoro
  modified_base 17..21: mod_base = OTHER; note = modified with 2'-methoxy
  modified_base 1..3: mod_base = OTHER; note = two adjacent nucleosides are linked by phosphorothioate diester groups
  modified_base 19..21: mod_base = OTHER; note = two adjacent nucleosides are linked by phosphorothioate diester groups
  modified_base 1: mod_base = OTHER; note = 5'-E-VP
tatacaactggctaaggggct

SEQ ID NO: 222 - RNA, 21 nt, Synthetic Construct
  source 1..21: mol_type = other RNA; note = modified anti-sense strand
  modified_base 1: mod_base = OTHER; note = modified with 2'-methoxy
  modified_base 2: mod_base = OTHER; note = modified with 2'-Fluoro
  modified_base 3..5: mod_base = OTHER; note = modified with 2'-methoxy
  modified_base 6: mod_base = OTHER; note = modified with 2'-Fluoro
  modified_base 7..11: mod_base = OTHER; note = modified with 2'-methoxy
  modified_base 12: mod_base = OTHER; note = modified with 2'-Fluoro
  modified_base 13: mod_base = OTHER; note = modified with 2'-methoxy
  modified_base 14: mod_base = OTHER; note = modified with 2'-Fluoro
  modified_base 15: mod_base = OTHER; note = modified with 2'-methoxy
  modified_base 16: mod_base = OTHER; note = modified with 2'-Fluoro
  modified_base 17..21: mod_base = OTHER; note = modified with 2'-methoxy
  modified_base 1..3: mod_base = OTHER; note = two adjacent nucleosides are linked by phosphorothioate diester groups
  modified_base 19..21: mod_base = OTHER; note = two adjacent nucleosides are linked by phosphorothioate diester groups
  modified_base 1: mod_base = OTHER; note = 5'-E-VP
tgaactcccacgttcacatga

SEQ ID NO: 223 - RNA, 21 nt, Synthetic Construct
  source 1..21: mol_type = other RNA; note = modified anti-sense strand
  modified_base 1: mod_base = OTHER; note = modified with 2'-methoxy
  modified_base 2: mod_base = OTHER; note = modified with 2'-Fluoro
  modified_base 3..5: mod_base = OTHER; note = modified with 2'-methoxy
  modified_base 6: mod_base = OTHER; note = modified with 2'-Fluoro
  modified_base 7..11: mod_base = OTHER; note = modified with 2'-methoxy
  modified_base 12: mod_base = OTHER; note = modified with 2'-Fluoro
  modified_base 13: mod_base = OTHER; note = modified with 2'-methoxy
  modified_base 14: mod_base = OTHER; note = modified with 2'-Fluoro
  modified_base 15: mod_base = OTHER; note = modified with 2'-methoxy
  modified_base 16: mod_base = OTHER; note = modified with 2'-Fluoro
  modified_base 17..21: mod_base = OTHER; note = modified with 2'-methoxy
  modified_base 1..3: mod_base = OTHER; note = two adjacent nucleosides are linked by phosphorothioate diester groups
  modified_base 19..21: mod_base = OTHER; note = two adjacent nucleosides are linked by phosphorothioate diester groups
  modified_base 1: mod_base = OTHER; note = 5'-E-VP
taagcatctgaaatacttaaa

SEQ ID NO: 224 - RNA, 21 nt, Synthetic Construct
  source 1..21: mol_type = other RNA; note = modified anti-sense strand
  modified_base 1: mod_base = OTHER; note = modified with 2'-methoxy
  modified_base 2: mod_base = OTHER; note = modified with 2'-Fluoro
  modified_base 3..5: mod_base = OTHER; note = modified with 2'-methoxy
  modified_base 6: mod_base = OTHER; note = modified with 2'-Fluoro
  modified_base 7..11: mod_base = OTHER; note = modified with 2'-methoxy
  modified_base 12: mod_base = OTHER; note = modified with 2'-Fluoro
  modified_base 13: mod_base = OTHER; note = modified with 2'-methoxy
  modified_base 14: mod_base = OTHER; note = modified with 2'-Fluoro
  modified_base 15: mod_base = OTHER; note = modified with 2'-methoxy
  modified_base 16: mod_base = OTHER; note = modified with 2'-Fluoro
  modified_base 17..21: mod_base = OTHER; note = modified with 2'-methoxy
  modified_base 1..3: mod_base = OTHER; note = two adjacent nucleosides are linked by phosphorothioate diester groups
  modified_base 19..21: mod_base = OTHER; note = two adjacent nucleosides are linked by phosphorothioate diester groups
  modified_base 1: mod_base = OTHER; note = 5'-E-VP
tgtgtatcctcttaattccta

SEQ ID NO: 225 - RNA, 21 nt, Synthetic Construct
  source 1..21: mol_type = other RNA; note = modified anti-sense strand
  modified_base 1: mod_base = OTHER; note = modified with 2'-methoxy
  modified_base 2: mod_base = OTHER; note = modified with 2'-Fluoro
  modified_base 3..5: mod_base = OTHER; note = modified with 2'-methoxy
  modified_base 6: mod_base = OTHER; note = modified with 2'-Fluoro
  modified_base 7..11: mod_base = OTHER; note = modified with 2'-methoxy
  modified_base 12: mod_base = OTHER; note = modified with 2'-Fluoro
  modified_base 13: mod_base = OTHER; note = modified with 2'-methoxy
  modified_base 14: mod_base = OTHER; note = modified with 2'-Fluoro
  modified_base 15: mod_base = OTHER; note = modified with 2'-methoxy
  modified_base 16: mod_base = OTHER; note = modified with 2'-Fluoro
  modified_base 17..21: mod_base = OTHER; note = modified with 2'-methoxy
  modified_base 1..3: mod_base = OTHER; note = two adjacent nucleosides are linked by phosphorothioate diester groups
  modified_base 19..21: mod_base = OTHER; note = two adjacent nucleosides are linked by phosphorothioate diester groups
  modified_base 1: mod_base = OTHER; note = 5'-E-VP
ttgtgtatcctcttaattcct

SEQ ID NO: 226 - RNA, 21 nt, Synthetic Construct
  source 1..21: mol_type = other RNA; note = modified anti-sense strand
  modified_base 1: mod_base = OTHER; note = modified with 2'-methoxy
  modified_base 2: mod_base = OTHER; note = modified with 2'-Fluoro
  modified_base 3..5: mod_base = OTHER; note = modified with 2'-methoxy
  modified_base 6: mod_base = OTHER; note = modified with 2'-Fluoro
  modified_base 7..11: mod_base = OTHER; note = modified with 2'-methoxy
  modified_base 12: mod_base = OTHER; note = modified with 2'-Fluoro
  modified_base 13: mod_base = OTHER; note = modified with 2'-methoxy
  modified_base 14: mod_base = OTHER; note = modified with 2'-Fluoro
  modified_base 15: mod_base = OTHER; note = modified with 2'-methoxy
  modified_base 16: mod_base = OTHER; note = modified with 2'-Fluoro
  modified_base 17..21: mod_base = OTHER; note = modified with 2'-methoxy
  modified_base 1..3: mod_base = OTHER; note = two adjacent nucleosides are linked by phosphorothioate diester groups
  modified_base 19..21: mod_base = OTHER; note = two adjacent nucleosides are linked by phosphorothioate diester groups
  modified_base 1: mod_base = OTHER; note = 5'-E-VP
tagcttgaagtctcaatgcct

SEQ ID NO: 227 - RNA, 21 nt, Synthetic Construct
  source 1..21: mol_type = other RNA; note = modified anti-sense strand
  modified_base 1: mod_base = OTHER; note = modified with 2'-methoxy
  modified_base 2: mod_base = OTHER; note = modified with 2'-Fluoro
  modified_base 3..5: mod_base = OTHER; note = modified with 2'-methoxy
  modified_base 6: mod_base = OTHER; note = modified with 2'-Fluoro
  modified_base 7..11: mod_base = OTHER; note = modified with 2'-methoxy
  modified_base 12: mod_base = OTHER; note = modified with 2'-Fluoro
  modified_base 13: mod_base = OTHER; note = modified with 2'-methoxy
  modified_base 14: mod_base = OTHER; note = modified with 2'-Fluoro
  modified_base 15: mod_base = OTHER; note = modified with 2'-methoxy
  modified_base 16: mod_base = OTHER; note = modified with 2'-Fluoro
  modified_base 17..21: mod_base = OTHER; note = modified with 2'-methoxy
  modified_base 1..3: mod_base = OTHER; note = two adjacent nucleosides are linked by phosphorothioate diester groups
  modified_base 19..21: mod_base = OTHER; note = two adjacent nucleosides are linked by phosphorothioate diester groups
  modified_base 1: mod_base = OTHER; note = 5'-E-VP
taagcttgaagtctcaatgcc

SEQ ID NO: 228 - RNA, 21 nt, Synthetic Construct
  source 1..21: mol_type = other RNA; note = modified anti-sense strand
  modified_base 1: mod_base = OTHER; note = modified with 2'-methoxy
  modified_base 2: mod_base = OTHER; note = modified with 2'-Fluoro
  modified_base 3..5: mod_base = OTHER; note = modified with 2'-methoxy
  modified_base 6: mod_base = OTHER; note = modified with 2'-Fluoro
  modified_base 7..11: mod_base = OTHER; note = modified with 2'-methoxy
  modified_base 12: mod_base = OTHER; note = modified with 2'-Fluoro
  modified_base 13: mod_base = OTHER; note = modified with 2'-methoxy
  modified_base 14: mod_base = OTHER; note = modified with 2'-Fluoro
  modified_base 15: mod_base = OTHER; note = modified with 2'-methoxy
  modified_base 16: mod_base = OTHER; note = modified with 2'-Fluoro
  modified_base 17..21: mod_base = OTHER; note = modified with 2'-methoxy
  modified_base 1..3: mod_base = OTHER; note = two adjacent nucleosides are linked by phosphorothioate diester groups
  modified_base 19..21: mod_base = OTHER; note = two adjacent nucleosides are linked by phosphorothioate diester groups
  modified_base 1: mod_base = OTHER; note = 5'-E-VP
tccagcagagcacccctcccc

SEQ ID NO: 229 - RNA, 19 nt, Synthetic Construct
  source 1..19: mol_type = other RNA; note = unmodified sense strand
gtctaccctgaactgcaga

SEQ ID NO: 230 - RNA, 19 nt, Synthetic Construct
  source 1..19: mol_type = other RNA; note = unmodified sense strand
gatgacgaggacgatgagg

SEQ ID NO: 231 - RNA, 19 nt, Synthetic Construct
  source 1..19: mol_type = other RNA; note = unmodified sense strand
gtgaacgtgggagttcagc

SEQ ID NO: 232 - RNA, 19 nt, Synthetic Construct
  source 1..19: mol_type = other RNA; note = unmodified sense strand
ttttaagtatttcagatgc

SEQ ID NO: 233 - RNA, 19 nt, Synthetic Construct
  source 1..19: mol_type = other RNA; note = unmodified sense strand
aggggtgctctgctggtct

SEQ ID NO: 234 - RNA, 21 nt, Synthetic Construct
  source 1..21: mol_type = other RNA; note = unmodified anti-sense strand
tctgcagttcagggtagactt

SEQ ID NO: 235 - RNA, 21 nt, Synthetic Construct
  source 1..21: mol_type = other RNA; note = unmodified anti-sense strand
cctcatcgtcctcgtcatcat

SEQ ID NO: 236 - RNA, 21 nt, Synthetic Construct
  source 1..21: mol_type = other RNA; note = unmodified anti-sense strand
gctgaactcccacgttcacat

SEQ ID NO: 237 - RNA, 21 nt, Synthetic Construct
  source 1..21: mol_type = other RNA; note = unmodified anti-sense strand
gcatctgaaatacttaaaaat

SEQ ID NO: 238 - RNA, 21 nt, Synthetic Construct
  source 1..21: mol_type = other RNA; note = unmodified anti-sense strand
agaccagcagagcacccctcc

SEQ ID NO: 239 - DNA, 20 bp, Synthetic Construct
  source 1..20: PCR_primers = fwd_name: hAPP, fwd_seq: gacagacagcacaccctaaa,rev_name: hAPP, rev_seq: cacacggaggtgtgtcataa; mol_type = other DNA
gacagacagcacaccctaaa

SEQ ID NO: 240 - DNA, 20 bp, Synthetic Construct
  source 1..20: PCR_primers = fwd_name: hAPP, fwd_seq: gacagacagcacaccctaaa,rev_name: hAPP, rev_seq: cacacggaggtgtgtcataa; mol_type = other DNA
cacacggaggtgtgtcataa

SEQ ID NO: 241 - DNA, 24 bp, Synthetic Construct
  source 1..24: mol_type = other DNA; note = hAPP-Probe
atcccaagaaagccgctcagatcc

SEQ ID NO: 242 - DNA, 24 bp, Synthetic Construct
  source 1..24: PCR_primers = fwd_name: hGAPDH, fwd_seq: gaccccttcattgacctcaactac,rev_name: hGAPDH, rev_seq: ttgacggtgccatggaattt; mol_type = other DNA
gaccccttcattgacctcaactac

SEQ ID NO: 243 - DNA, 20 bp, Synthetic Construct
  source 1..20: PCR_primers = fwd_name: hGAPDH, fwd_seq: gaccccttcattgacctcaactac,rev_name: hGAPDH, rev_seq: ttgacggtgccatggaattt; mol_type = other DNA
ttgacggtgccatggaattt

SEQ ID NO: 244 - DNA, 22 bp, Synthetic Construct
  source 1..22: mol_type = other DNA; note = hGAPDH-Probe
ttacatgttccaatatgattcc

SEQ ID NO: 245 - DNA, 21 bp, Synthetic Construct
  source 1..21: PCR_primers = fwd_name: mkAPP, fwd_seq: cccactttgtgattccctacc,rev_name: mkAPP, rev_seq: atccatcctctcctggtgtaa; mol_type = other DNA
cccactttgtgattccctacc

SEQ ID NO: 246 - DNA, 21 bp, Synthetic Construct
  source 1..21: PCR_primers = fwd_name: mkAPP, fwd_seq: cccactttgtgattccctacc,rev_name: mkAPP, rev_seq: atccatcctctcctggtgtaa; mol_type = other DNA
atccatcctctcctggtgtaa

SEQ ID NO: 247 - DNA, 27 bp, Synthetic Construct
  source 1..27: mol_type = other DNA; note = mkAPP-Probe
tagttggtgagtttgtaagcgatgccc

SEQ ID NO: 248 - DNA, 20 bp, Synthetic Construct
  source 1..20: PCR_primers = fwd_name: mkGAPDH, fwd_seq: tcaagatcgtcagcaacgcc,rev_name: mkGAPDH, rev_seq: acagtcttctgggtggcagt; mol_type = other DNA
tcaagatcgtcagcaacgcc

SEQ ID NO: 249 - DNA, 20 bp, Synthetic Construct
  source 1..20: PCR_primers = fwd_name: mkGAPDH, fwd_seq: tcaagatcgtcagcaacgcc,rev_name: mkGAPDH, rev_seq: acagtcttctgggtggcagt; mol_type = other DNA
acagtcttctgggtggcagt

SEQ ID NO: 250 - DNA, 25 bp, Synthetic Construct
  source 1..25: mol_type = other DNA; note = mkGAPDH-Probe
accaactgcttagcacccctggcca